European Patent Specification EP 2 875 047 B1, published January 25, 2023. Title: Production Cell Line Enhancers. Applicant: Regeneron Pharmaceuticals, Inc. The sequence listing filed with the application follows.

SEQUENCE LISTING (46 sequences)

SEQ ID NO: 1 - protein, 577 aa, Mus musculus
MPFRLLIPLGLVCVLLPLHHGAPGPDGTAPDPAHYRERVKAMFYHAYDSYLENAFPYDELRPLTCDGHDTWGSFSLTLIDALDTLLILGNTSEFQRVVEVLQDNVDFDIDVNASVFETNIRVVGGLLSAHLLSKKAGVEVEAGWPCSGPLLRMAEEAARKLLPAFQTPTGMPYGTVNLLHGVNPGETPVTCTAGIGTFIVEFATLSSLTGDPVFEDVARVALMRLWESRSDIGLVGNHIDVLTGKWVAQDAGIGAGVDSYFEYLVKGAILLQDKKLMAMFLEYNKAIRNYTHFDDWYLWVQMYKGTVSMPVFQSLEAYWPGLQSLIGDIDNAMRTFLNYYTVWKQFGGLPEFYNIPQGYTVEKREGYPLRPELIESAMYLYRATGDPTLLELGRDAVESIEKISKVECGFATIKDLRDHKLDNRMESFFLAETVKYLYLLFHPNNFIHNNGSTFDSVMTPHGECILGAGGYIFNTEAHPIDPAALHCCRRLKEEQWEVEDLIKEFYSLKQSRPKRAQRKTVRSGPWEPQSGPATLSSPANQPREKQPAQQRTPLLSCPSQPFTSKLALLGQVFLDSS

SEQ ID NO: 2 - protein, 576 aa, Rattus norvegicus
MPFRLLIPLGLVCVLLPLHHGAPGPEGTAPDPAHYRERVKAMFYHAYDSYLENAFPYDELRPLTCDGHDTWGSFSLTLIDALDTLLILGNTSEFQRVVEVLQDNVDFDIDVNASVFETNIRVVGGLLSAHLLSKKAGVEVEAGWPCSGPLLRMAEEAARKLLPAFQTPTGMPYGTVNLLHGVNPGETPVTCTAGIGTFIVEFATLSSLTGDPVFEDVARVALMRLWESRSDIGLVGNHIDVLTGKWVAQDAGIGAGVDSYFEYLVKGAILLQDKKLMAMFLEYNKAIRNYTHFDDWYLWVQMYKGTVSMPVFQSLEAYWPGLQSLIGDIDNAMRTFLNYYTVWKQFGGLPEFYNIPQGYTVEKREGYPLRPELIESAMYLYRATGDPTLLELGRDAVESIEKISKVECGFATIKDLRDHKLDNRMESFFLAETVKYLYLLFHPNNFIHNNGSTFDSVMTPHGECILGAGGYIFNTEAHPIDPAALHCCRRLKEEQWEVEDLIKEFYSLRQSRSRAQRKTVSSGPWEPPAGPGTLSSPENQPREKQPARQRAPLLSCPSQPFTSKLALLGQVFLDSS

SEQ ID NO: 3 - protein, 578 aa, Cricetulus griseus
MPFRLLIPLGLVCVFLPLHHGAPGPDGTAPDPAHYRERVKAMFYHAYDSYLENAFPYDELRPLTCDGHDTWGSFSLTLIDALDTLLILGNTSEFQRVVEVLQDNVDFDIDVNASVFETNIRVVGGLLSAHLLSKKAGVEVEAGWPCSGPLLRMAEEAARKLLPAFQTPTGMPYGTVNLLHGVNPGETPVTCTAGIGTFIVEFATLSSLTGDPVFEDVARLALMRLWESRSDIGLVGNHIDVLTGKWVAQDAGIGAGVDSYFEYLVKGAILLQDKKLMAMFLEYNRAIRNYTHFDDWYLWVQMYKGTVSMPVFQSLEAYWPGLQSLIGDIDNAMRTFLNYYTVWKQFGGLPEFYNIAQGYTVEKREGYPLRPELIESAMYLYRATGDPTLLELGRDAVESIEKISKVECGFATIKDLRDHKLDNRMESFFLAETVKYLYLLFHPNNFIHNNGSTFDSVMTPHGECILGAGGYIFNTEAHPIDPAALHCCRRLKEEQWEVEDLMRELHSLKQSRSRAQRKTTSSGPWEPPAGPGSPSAPGKQDQPREKQPAKQRTPLLSCPSQPFTSKLALLGQVFLDSS

SEQ ID NO: 4 - protein, 578 aa, Homo sapiens [sequence omitted]

SEQ ID NO: 5 - protein, 578 aa, Pan troglodytes
MPFRLLIPLGLLCALLPLHHGAPGPDGSAPDPAHYRERVKAMFYHAYDSYLENAFPFDELRPLTCDGHDTWGSFSLTLIDALDTLLILGNVSEFQRVVEVLQDSVDFDIDVNASVFETNIRVVGGLLSAHLLSKKAGVEVEAGWPCSGPLLRMAEEAARKLLPAFQTPTGMPYGTVNLLHGVNPGETPVTCTAGIGTFIVEFATLSSLTGDPVFEDVARVALMRLWESRSDIGLVGNHIDVLTGKWVAQDAGIGAGVDSYFEYLVKGAILLQDKKLMAMFLEYNKAIRNYTRFDDWYLWVQMYKGTVSMPVFQSLEAYWPGLQSLIGDIDNAMRTFLNYYTVWKQFGGLPEFYNIPQGYTVEKREGYPLRPELIESAMYLYRATGDPTLLELGRDAVESIEKISKVECGFATIKDLRDHKLDNRMESFFLAETVKYLYLLFDPTNFIHNNGSTFDAVITPYGECILGAGGYIFNTEAHPIDPAALHCCQRLKEEQWEVEDLMREFYSLKRSRSKFQKKTVSSGPWEPPARPGTLFSPENHDQARERKPAKQKVPLLSCPSQPFTSKLALLGQVFLDSS

SEQ ID NO: 6 - protein, 513 aa, Pongo pygmaeus
MNTLSCSLFSLTLIDALDTLLILGNVSEFQRVVEVLQDNVDFDIDVNASVFETNIRVVGGLLSAHLLSKKAGVEVEAGWPCSGPLLRMAEEAARKLLPAFQTPTGMPYGTVNLLHGVNPGETPVTCTAGIGTFIVEFATLSSLTGDPVFEDVARVALMRLWESRSDIGLVGNHIDVLTGKWVAQDAGIGAGVDSYFEYLVKGAILLQDKKLMAMFLEYNKAIRNYTRFDDWYLWVQMYKGTVSMPVFQSLEAYWPGLQSLIGDIDNAMRTFLNYYTVWKQFGGLPEFYNIPQGYTVEKREGYPLRPELIESAMYLYRATGDPTLLELGRDAVESIEKISKVECGFATIKDLRDHKLDNRMESFFLAETVKYLYLLFDPTNFIHNNGSTFDAVITPYGECILGAGGYIFNTEAHPIDPAALHCCQRLKEEQWEVEDLMREFYSLKRNRSKFQKKTVSSGPWEPPARPGTLFSPENHDQARGRKPAKQKVPLLSCPSQPFTSKLALLGQVFLDSS

SEQ ID NO: 7 - protein, 572 aa, Danio rerio
LYYLPLFTSRYFMLTFLFSAIFCAAYLSPIISHVKGRDFTEQEMSHYRDRVKSMFYHAYNSYLDNAYPYDELRPLTCDGQDTWGSFSLTLIDALDTLLILGNHTEFQRVATLLQDTVDFDIDVNASVFETNIRVVGGLLSAHLLSKRAGMKVEEGWPCSGPLLRMAEDAARKLLPAFQTPTGMPYGTVNLLRGVNPGETPVTCTAGVGTFILEFSTLSRLTGDPVFENVARKALRALWRTRSDIGLVGNHIDVITSKWVAQDAGIGAGVDSYFEYLVRGAIMLQDEELLTMFYEFDKSIKNYTKFDDWYLWVQMHKGTVSMPVFQSLEAFWPGMQSLIGDISSATKSFHNYYSVWRQFGGLPEFYSIPQGYTVDKREGYPLRPELIESAMYLYKATGDPSFIQLGRDAVESIDRISRVNCGFATVKDVRDHKLDNRMESFFLAETIKYLYLLFDPDNFLHNTGTEFELGGLRGDCILSAGGYVFNTEAHPLDPAALHCCSREQQDRREIQDILLSFSQPHTEEPSRDQSAGGSPESIALKPGEQRKAPVLSCPTQPFSAKLAVMGQVFSDNS

SEQ ID NO: 8 - protein, 577 aa, Artificial
  Consensus sequence
  MISC_FEATURE (12)..(12): V or L
  MISC_FEATURE (14)..(14): V or A
  MISC_FEATURE (15)..(15): L or F
  MISC_FEATURE (26)..(26): D or E
  MISC_FEATURE (28)..(28): T or S
  MISC_FEATURE (57)..(57): Y or F
  MISC_FEATURE (91)..(91): T or V
  MISC_FEATURE (104)..(104): N or S
  MISC_FEATURE (220)..(220): V or L
  MISC_FEATURE (285)..(285): K or R
  MISC_FEATURE (292)..(292): H or R
  MISC_FEATURE (356)..(356): P or A
  MISC_FEATURE (442)..(442): H or D
  MISC_FEATURE (444)..(444): N or T
  MISC_FEATURE (456)..(456): S, T, or A
  MISC_FEATURE (458)..(458): M or I
  MISC_FEATURE (461)..(461): H or Y
  MISC_FEATURE (489)..(489): R or Q
  MISC_FEATURE (502)..(502): I or M
  MISC_FEATURE (503)..(503): K or R
  MISC_FEATURE (505)..(505): F or L
  MISC_FEATURE (506)..(506): Y or H
  MISC_FEATURE (509)..(509): K or R
  MISC_FEATURE (510)..(510): Q or R
  MISC_FEATURE (513)..(513): P or S
  MISC_FEATURE (514)..(516): KRA, RA, or KF
  MISC_FEATURE (518)..(518): R or K
  MISC_FEATURE (519)..(519): K or N
  MISC_FEATURE (522)..(522): R or S
  MISC_FEATURE (529)..(529): Q or P
  MISC_FEATURE (530)..(530): S or A
  MISC_FEATURE (531)..(531): G or R
  MISC_FEATURE (533)..(533): A or G
  MISC_FEATURE (534)..(534): T or S
  MISC_FEATURE (535)..(535): L or P
  MISC_FEATURE (536)..(536): S or F
  MISC_FEATURE (537)..(537): S or A
  MISC_FEATURE (539)..(540): AN, EN, GKQD, or ENHD
  MISC_FEATURE (542)..(542): P or A
  MISC_FEATURE (545)..(545): K or R
  MISC_FEATURE (546)..(546): Q or K
  MISC_FEATURE (549)..(549): Q, R, or K
  MISC_FEATURE (551)..(551): R or K
  MISC_FEATURE (552)..(552): T, A, or V
MPFRLLIPLGLXCXXLPLHHGAPGPXGXAPDPAHYRERVKAMFYHAYDSYLENAFPXDELRPLTCDGHDTWGSFSLTLIDALDTLLILGNXSEFQRVVEVLQDXVDFDIDVNASVFETNIRVVGGLLSAHLLSKKAGVEVEAGWPCSGPLLRMAEEAARKLLPAFQTPTGMPYGTVNLLHGVNPGETPVTCTAGIGTFIVEFATLSSLTGDPVFEDVARXALMRLWESRSDIGLVGNHIDVLTGKWVAQDAGIGAGVDSYFEYLVKGAILLQDKKLMAMFLEYNXAIRNYTXFDDWYLWVQMYKGTVSMPVFQSLEAYWPGLQSLIGDIDNAMRTFLNYYTVWKQFGGLPEFYNIXQGYTVEKREGYPLRPELIESAMYLYRATGDPTLLELGRDAVESIEKISKVECGFATIKDLRDHKLDNRMESFFLAETVKYLYLLFXPXNFIHNNGSTFDXVXTPXGECILGAGGYIFNTEAHPIDPAALHCCXRLKEEQWEVEDLXXEXXSLXXSRXXXXQXXTVXSGPWEPXXXPXXXXXPXXQXREXXPAXQXXPLLSCPSQPFTSKLALLGQVFLDSS

SEQ ID NO: 9 - protein, 371 aa, Mus musculus
MVVVAAAPSAATAAPKVLLLSGQPASGGRALPLMVPGPRAAGSEASGTPQARKRQRLTHLSPEEKALRRKLKNRVAAQTARDRKKARMSELEQQVVDLEEENHKLQLENQLLREKTHGLVVENQELRTRLGMDTLDPDEVPEVEAKGSGVRLVAGSAESAAGAGPVVTSPEHLPMDSDTVASSDSESDILLGILDKLDPVMFFKCPSPESASLEELPEVYPEGPSSLPASLSLSVGTSSAKLEAINELIRFDHVYTKPLVLEIPSETESQTNVVVKIEEAPLSSSEEDHPEFIVSVKKEPLEDDFIPELGISNLLSSSHCLRPPSCLLDAHSDCGYEGSPSPFSDMSSPLGTDHSWEDTFANELFPQLISV

SEQ ID NO: 10 - protein, 369 aa, Cricetulus griseus
MVVVAASPSAATAAPKVLLLSGQPAADGRALPLMVPGSRAAGSEANGAPQARKRQRLTHLSPEEKALRRKLKNRVAAQTARDRKKARMSELEQQVVDLEEENQKLLLENQLLREKTHGLVIENQELRTRLGMDVLTTEEAPETESKGNGVRPVAGSAESAAGAGPVVTSPEHLPMDSDTVDSSDSESDILLGILDKLDPVMFFKCPSPESANLEELPEVYPGPSSLPASLSLSVGTSSAKLEAINELIRFDHVYTKPLVLEIPSETESQTNVVVKIEEAPLSSSEEDHPEFIVSVKKEPEEDFIPEPGISNLLSSSHCLKPSSCLLDAYSDCGYEGSPSPFSDMSSPLGIDHSWEDTFANELFPQLISV

SEQ ID NO: 11 - protein, 376 aa, Homo sapiens
MVVVAAAPNPADGTPKVLLLSGQPASAAGAPAGQALPLMVPAQRGASPEAASGGLPQARKRQRLTHLSPEEKALRRKLKNRVAAQTARDRKKARMSELEQQVVDLEEENQKLLLENQLLREKTHGLVVENQELRQRLGMDALVAEEEAEAKGNEVRPVAGSAESAAGAGPVVTPPEHLPMDSGGIDSSDSESDILLGILDNLDPVMFFKCPSPEPASLEELPEVYPEGPSSLPASLSLSVGTSSAKLEAINELIRFDHIYTKPLVLEIPSETESQANVVVKIEEAPLSPSENDHPEFIVSVKEEPVEDDLVPELGISNLLSSSHCPKPSSCLLDAYSDCGYGGSLSPFSDMSSLLGVNHSWEDTFANELFPQLISV

SEQ ID NO: 12 - protein, 383 aa, Danio rerio
MVVVTAGTGGAHKVLLISGKQSASTGATQGGYSRSISVMIPNQASSDSDSTTSGPPLRKRQRLTHLSPEEKALRRKLKNRVAAQTARDRKKAKMGELEQQVLELELENQKLHVENRLLRDKTSDLLSENEELRQRLGLDTLETKEQVQVLESAVSDLGLVTGSSESAAGAGPAVPKSEDFTMDTHSPGPADSESDLLLGILDILDPELFLKTDLPEAQEPQQELVLVGGAGEQVPSSAPAALGPAPVKLEALNELIHFDHIYTKPAEVLVSEESICEVKAEDSVAFSETEEEIQVEDQTVSVKDEPEEVVIPAENQNPDAADDFLSDTSFGGYEKASYLTDAYSDSGYERSPSPFSNISSPLCSEGSWDDMFASELFPQLISV

SEQ ID NO: 13 - protein, 371 aa, Artificial
  consensus sequence
  MISC_FEATURE (7)..(7): A or S
  MISC_FEATURE (9)..(9): S or N
  MISC_FEATURE (10)..(10): A or P
  MISC_FEATURE (12)..(12): T or D
  MISC_FEATURE (13)..(13): A or G
  MISC_FEATURE (14)..(14): A or T
  MISC_FEATURE (26)..(26): S or A
  misc_feature (27)..(27): Xaa can be any naturally occurring amino acid
  MISC_FEATURE (29)..(29): R or Q
  MISC_FEATURE (37)..(37): G or A
  misc_feature (38)..(38): Xaa can be any naturally occurring amino acid
  MISC_FEATURE (40)..(40): A or G
  MISC_FEATURE (46)..(46): S or N, or ASG
  MISC_FEATURE (48)..(48): T, A, or L
  MISC_FEATURE (103)..(103): H or Q
  MISC_FEATURE (106)..(106): Q or L
  MISC_FEATURE (121)..(121): V or I
  MISC_FEATURE (128)..(128): T or Q
  MISC_FEATURE (134)..(134): T, V, or A
  MISC_FEATURE (136)..(136): D, T, or V
  MISC_FEATURE (137)..(137): P, T, or A
  MISC_FEATURE (138)..(138): D or E
  MISC_FEATURE (140)..(140): V, A, or none
  MISC_FEATURE (141)..(141): P or none
  MISC_FEATURE (143)..(143): V, T, or A
  MISC_FEATURE (145)..(145): A or S
  MISC_FEATURE (148)..(148): S or N
  MISC_FEATURE (149)..(149): G or E
  MISC_FEATURE (152)..(152): L or P
  MISC_FEATURE (169)..(169): S or P
  MISC_FEATURE (178)..(178): D or G
  MISC_FEATURE (179)..(179): T or G
  MISC_FEATURE (180)..(180): V or I
  MISC_FEATURE (181)..(181): A or D
  MISC_FEATURE (196)..(196): K or N
  MISC_FEATURE (210)..(210): S or P
  MISC_FEATURE (212)..(212): S or N
  MISC_FEATURE (222)..(222): E or none
  MISC_FEATURE (254)..(254): V or I
  MISC_FEATURE (271)..(271): T or A
  MISC_FEATURE (284)..(284): S or P
  MISC_FEATURE (287)..(287): E or N
  MISC_FEATURE (298)..(298): K or E
  MISC_FEATURE (301)..(301): L, V, or none
  MISC_FEATURE (303)..(303): D or E
  MISC_FEATURE (305)..(305): F or L
  MISC_FEATURE (306)..(306): I or V
  MISC_FEATURE (309)..(309): L or P
  MISC_FEATURE (321)..(321): L or P
  MISC_FEATURE (322)..(322): R or K
  MISC_FEATURE (324)..(324): P or S
  MISC_FEATURE (331)..(331): H or Y
  MISC_FEATURE (337)..(337): E or G
  MISC_FEATURE (340)..(340): P or L
  MISC_FEATURE (349)..(349): P or L
  MISC_FEATURE (352)..(352): T, I, or V
  MISC_FEATURE (353)..(353): D or N
MVVVAAXPXXAXXXPKVLLLSGQPAXXGRALPLMVPXXRXAGSEAXGXPQARKRQRLTHLSPEEKALRRKLKNRVAAQTARDRKKARMSELEQQVVDLEEENXKLXLENQLLREKTHGLVXENQELRXRLGMDXLDXXEXXEXEXKGXXVRXVAGSAESAAGAGPVVTXPEHLPMDSXXXXSSDSESDILLGILDXLDPVMFFKCPSPEXAXLEELPEVYPXGPSSLPASLSLSVGTSSAKLEAINELIRFDHXYTKPLVLEIPSETESQXNVVVKIEEAPLSXSEXDHPEFIVSVKXEPXEXDXXPEXGISNLLSSSHCXXPXSCLLDAXSDCGYXGSXSPFSDMSSXLGXXHSWEDTFANELFPQLISV

SEQ ID NO: 14 - DNA, 7686 bp, Artificial
  Synthetic plasmid
aagcttatactcgagctctagattgggaacccgggtctctcgaattcgatgccttttagactcctgataccattgggtcttgtttgcgttctcctccctctccatcacggcgccccaggtccagacggtaccgcacctgatcctgcccattaccgcgaacgcgttaaagccatgttctaccacgcctatgactcctatctggaaaatgcattcccctatgatgagctccgaccccttacctgcgatggtcatgatacttggggctctttttcccttacccttattgacgctctggacacactccttatcctcggaaacaccagcgaatttcaaagagtagttgaagtacttcaggacaatgtcgactttgacatcgatgtgaacgcatcagttttcgaaacaaatataagagtcgttggaggtctgctctccgcccaccttctctctaaaaaagccggagtagaagttgaagctggctggccctgctccggacccctccttcgtatggctgaagaagctgcccgcaaactccttcccgcttttcagaccccaaccggtatgccctatggtactgttaacctcctgcacggagtaaatcccggcgaaacccccgtcacatgtacagccggaattggaacctttattgtggaatttgcaacccttagcagcctgaccggagatcctgtattcgaagacgtggctcgggttgccctgatgcgactgtgggaatccaggtctgatatcggtctggtcggtaaccatatagacgtactcactggtaaatgggttgcacaagacgctggaattggggcaggcgtggattcttattttgaatatctcgtaaaaggggccatactcttgcaggacaaaaaacttatggctatgttcctggaatataacaaagctattaggaactacacacacttcgatgattggtatttgtgggtccaaatgtataaaggaaccgtttctatgcctgtctttcagtcactggaggcttattggcctggtctgcaatccctgatcggagacattgacaatgcaatgaggacattccttaattattacactgtttggaagcagttcggcggattgcccgaattttacaacattcctcaaggctatacagttgaaaaaagagaaggatatcccctgcgccccgagcttattgaaagcgctatgtatctgtatcgtgcaacaggtgatccaaccctgcttgaactgggacgagacgccgtcgaatcaatcgagaaaatttcaaaagtggaatgcggctttgcaacaattaaagatcttagagaccacaaactggataatcgcatggagtcattctttttggctgagaccgtcaagtatctgtatctgctttttcatcccaacaacttcatccataataacgggtccaccttcgattcagtcatgacccctcacggtgaatgcatactcggagctggaggctatatttttaacactgaagctcacccaattgacccagctgcccttcattgttgtcgacgtctgaaagaagaacaatgggaggttgaagatttgatcaaagaattttactcacttaaacaaagtcgacctaaacgcgcacagagaaaaactgtaagatctggtccttgggaacctcagtccggcccagcaactctttcatcccccgccaaccaaccacgagaaaaacaaccagcccaacagagaacccccctgctcagctgcccctctcagcccttcacttcaaaactcgccctgcttggacaggtgtttctggactcctcttgatttaaacacgcggccgctaatcagccataccacatttgtagaggttttacttgctttaaaaaacctcccacacctccccctgaacctgaaacataaaatgaatgcaattgttgttgttaacttgtttattgcagcttataatggttacaaataaagcaatagcatcacaaatttcacaaataaagcatttttttcactgcattctagttgtggtttgtccaaactcatcaatgtatcttatcatgtctaccggtagggcccctctcttcatgtgagcaaaaggccagcaaaaggccaggaaccgtaaaaaggccgcgttgctggcgtttttccataggctccgcccccctgacgagcatcacaaaaatcgacgctcaagtcagaggtggcgaaacccgacaggactataaagataccaggcgtttccccctggaagctccctcgtgcgctctcctgttccgaccctgccgcttaccggatacctgtccgcctttctcccttcgggaagcgtggcgctttctcaatgctcacgctgtaggtatctcagttcggtgtaggtcgttcgctccaagctgggctgtgtgcacgaaccccccgttcagcccgaccgctgcgccttatccggtaactatcgtcttgagtccaacccggtaagacacgacttatcgccactggcagcagccactggtaacaggattagcagagcgaggtatgtaggcggtgctacagagttcttgaagtggtggcctaactacggctacactagaaggacagtatttggtatctgcgctctgctgaagccagttaccttcggaaaaagagttggtagctcttgatccggcaaacaaaccaccgctggtagcggtggtttttttgtttgcaagcagcagattacgcgcagaaaaaaaggatctcaagaagatcctttgatcttttctacggggtctgacgctcagtggaacgaaaactcacgttaagggattttggtcatgggcgcgcctcatactcctgcaggcatgagattatcaaaaaggatcttcacctagatccttttaaattaaaaatgaagttttaaatcaatctaaagtatatatgagtaaacttggtctgacagttaccaatgcttaatcagtgaggcacctatctcagcgatctgtctatttcgttcatccatagttgcctgactccccgtcgtgtagataactacgatacgggagggcttaccatctggccccagtgctgcaatgataccgcgagacccacgctcaccggctccagatttatcagcaataaaccagccagccggaagggccgagcgcagaagtggtcctgcaactttatccgcctccatccagtctattaattgttgccgggaagctagagtaagtagttcgccagttaatagtttgcgcaacgttgttgccattgctacaggcatcgtggtgtcacgctcgtcgtttggtatggcttcattcagctccggttcccaacgatcaaggcgagttacatgatcccccatgttgtgcaaaaaagcggttagctccttcggtcctccgatcgttgtcagaagtaagttggccgcagtgttatcactcatggttatggcagcactgcataattctcttactgtcatgccatccgtaagatgcttttctgtgactggtgagtactcaaccaagtcattctgagaatagtgtatgcggcgaccgagttgctcttgcccggcgtcaatacgggataataccgcgccacatagcagaactttaaaagtgctcatcattggaaaacgttcttcggggcgaaaactctcaaggatcttaccgctgttgagatccagttcgatgtaacccactcgtgcacccaactgatcttcagcatcttttactttcaccagcgtttctgggtgagcaaaaacaggaaggcaaaatgccgcaaaaaagggaataagggcgacacggaaatgttgaatactcatactcttcctttttcaatattattgaagcatttatcagggttattgtctcatgagcggatacatatttgaatgtatttagaaaaataaacaaataggggttccgcgcacatttccccgaaaagtgccacctgacgtcaggtaccaagcctaggcctccaaaaaagcctcctcactacttctggaatagctcagaggcagaggcggcctcggcctctgcataaataaaaaaaattagtcagccatggggcggagaatgggcggaactgggcggagttaggggcgggatgggcggagttaggggcgggactatggttgctgactaattgagatgcatgctttgcatacttctgcctgctggggagcctggggactttccacacctggttgctgactaattgagatgcatgctttgcatacttctgcctgctggggagcctggggactttccacaccggatccaccatgggatcggccattgaacaagatggattgcacgcaggttctccggccgcttgggtggagaggctattcggctatgactgggcacaacagacaatcggctgctctgatgccgccgtgttccggctgtcagcgcaggggcgcccggttctttttgtcaagaccgacctgtccggtgccctgaatgaactgcaggacgaggcagcgcggctatcgtggctggccacgacgggcgttccttgcgcagctgtgctcgacgttgtcactgaagcgggaagggactggctgctattgggcgaagtgccggggcaggatctcctgtcatctcaccttgctcctgccgagaaagtatccatcatggctgatgcaatgcggcggctgcatacgcttgatccggctacctgcccattcgaccaccaagcgaaacatcgcatcgagcgagcacgtactcggatggaagccggtcttgtcgatcaggatgatctggacgaagagcatcaggggctcgcgccagccgaactgttcgccaggctcaaggcgcgcatgcccgacggcgatgatctcgtcgtgacccatggcgatgcctgcttgccgaatatcatggtggaaaatggccgcttttctggattcatcgactgtggccggctgggtgtggcggaccgctatcaggacatagcgttggctacccgtgatattgctgaagagcttggcggcgaatgggctgaccgcttcctcgtgctttacggtatcgccgctcccgattcgcagcgcatcgccttctatcgccttcttgacgagttcttctgaacgcgtgctgtaagtctgcagaaattgatgatctattaaacaataaagatgtccactaaaatggaagtttttcctgtcatactttgttaagaagggtgagaacagagtacctacattttgaatggaaggattggagctacgggggtgggggtggggtgggattagataaatgcctgctctttactgaaggctctttactattgctttatgataatgtttcatagttggatatcataatttaaacaagcaaaaccaaattaagggccagctcattcctcccactcatgatctatggatctatagatctctcgtgcagctggggctctagggggtatccccacgcgccctgtagcggcgcattaagcgcggcgggtgtggtggttacgcgcagcgtgaccgctacacttgccagcgccctagcgcccgctcctttcgctttcttcccttcctttctcgccacgttcgccggctttccccgtcaagctctaaatcgggggctccctttagggttccgatttagtgctttacggcacctcgaccccaaaaaacttgattagggtgatggttcacgtagtgggccatcgccctgatagacggtttttcgccctttgacgttggagtccacgttctttaatagtggactcttgttccaaactggaacaacactcaaccctatctcggtctattcttttgatttataagggattttgccgatttcggcctattggttaaaaaatgagctgatttaacaaaaatttaacgcgaattaattctgtggaatgtgtgtcagttagtcgcgaggcctccgcgccgggttttggcgcctcccgcgggcgcccccctcctcacggcgagcgctgccacgtcagacgaagggcgcagcgagcgtcctgatccttccgcccggacgctcaggacagcggcccgctgctcataagactcggccttagaaccccagtatcagcagaaggacattttaggacgggacttgggtgactctagggcactggttttctttccagagagcggaacaggcgaggaaaagtagtcccttctcggcgattctgcggagggatctccgtggggcggtgaacgccgatgattatataaggacgcgccgggtgtggcacagctagttccgtcgcagccgggatttgggtcgcggttcttgtttgtggatcgctgtgatcgtcacttggtgagtagcgggctgctgggctggccggggctttcgtggccgccgggccgctcggtgggacggaagcgtgtggagagaccgccaagggctgtagtctgggtccgcgagcaaggttgccctgaactgggggttggggggagcgcagcaaaatggcggctgttcccgagtcttgaatggaagacgcttgtgaggcgggctgtgaggtcgttgaaacaaggtggggggcatggtgggcggcaagaacccaaggtcttgaggccttcgctaatgcgggaaagctcttattcgggtgagatgggctggggcaccatctggggaccctgacgtgaagtttgtcactgactggagaactcggtttgtcgtctgttgcgggggcggcagttatggcggtgccgttgggcagtgcacccgtacctttgggagcgcgcgccctcgtcgtgtcgtgacgtcacccgttctgttggcttataatgcagggtggggccacctgccggtaggtgtgcggtaggcttttctccgtcgcaggacgcagggttcgggcctagggtaggctctcctgaatcgacaggcgccggacctctggtgaggggagggataagtgaggcgtcagtttctttggtcggttttatgtacctatcttcttaagtagctgaagctccggttttgaactatgcgctcggggttggcgagtgtgttttgtgaagttttttaggcaccttttgaaatgtaatcatttgggtcaatatgtaattttcagtgttagactagtaaattgtccgctaaattctggccgtttttggcttttttgttagacgtcgaccgatcctgagaacttcagggtgagtttggggacccttgattgttctttctttttcgctattgtaaaattcatgttatatggagggggcaaagttttcagggtgttgtttagaatgggaagatgtcccttgtatcaccatggaccctcatgataattttgtttctttcactttctactctgttgacaaccattgtctcctcttattttcttttcattttctgtaactttttcgttaaactttagcttgcatttgtaacgaatttttaaattcacttttgtttatttgtcagattgtaagtactttctctaatcacttttttttcaaggcaatcagggtatattatattgtacttcagcacagttttagagaacaattgttataattaaatgataaggtagaatatttctgcatataaattctggctggcgtggaaatattcttattggtagaaacaactacaccctggtcatcatcctgcctttctctttatggttacaatgatatacactgtttgagatgaggataaaatactctgagtccaaaccgggcccctctgctaaccatgttcatgccttcttctctttcctacagctcctgggcaacgtgctggttgttgtgctgtctcatcattttggcaaagaatt

SEQ ID NO: 15 - DNA, 7257 bp, Artificial
  Synthetic plasmid
aagcttatactcgagctctagattgggaacccgggtctctcgaattcgatgccttttagactcctgataccattgggtcttgtttgcgttctcctccctctccatcacggcgccccaggtccagacggtaccgcacctgatcctgcccattaccgcgaacgcgttaaagccatgttctaccacgcctatgactcctatctggaaaatgcattcccctatgatgagctccgaccccttacctgcgatggtcatgatacttggggctctttttcccttacccttattgacgctctggacacactccttatcctcggaaacaccagcgaatttcaaagagtagttgaagtacttcaggacaatgtcgactttgacatcgatgtgaacgcatcagttttcgaaacaaatataagagtcgttggaggtctgctctccgcccaccttctctctaaaaaagccggagtagaagttgaagctggctggccctgctccggacccctccttcgtatggctgaagaagctgcccgcaaactccttcccgcttttcagaccccaaccggtatgccctatggtactgttaacctcctgcacggagtaaatcccggcgaaacccccgtcacatgtacagccggaattggaacctttattgtggaatttgcaacccttagcagcctgaccggagatcctgtattcgaagacgtggctcgggttgccctgatgcgactgtgggaatccaggtctgatatcggtctggtcggtaaccatatagacgtactcactggtaaatgggttgcacaagacgctggaattggggcaggcgtggattcttattttgaatatctcgtaaaaggggccatactcttgcaggacaaaaaacttatggctatgttcctggaatataacaaagctattaggaactacacacacttcgatgattggtatttgtgggtccaaatgtataaaggaaccgtttctatgcctgtctttcagtcactggaggcttattggcctggtctgcaatccctgatcggagacattgacaatgcaatgaggacattccttaattattacactgtttggaagcagttcggcggattgcccgaattttacaacattcctcaaggctatacagttgaaaaaagagaaggatatcccctgcgccccgagcttattgaaagcgctatgtatctgtatcgtgcaacaggtgatccaaccctgcttgaactgggacgagacgccgtcgaatcaatcgagaaaatttcaaaagtggaatgcggctttgcaacaattaaagatcttagagaccacaaactggataatcgcatggagtcattctttttggctgagaccgtcaagtatctgtatctgctttttcatcccaacaacttcatccataataacgggtccaccttcgattcagtcatgacccctcacggtgaatgcatactcggagctggaggctatatttttaacactgaagctcacccaattgacccagctgcccttcattgttgtcgacgtctgaaagaagaacaatgggaggttgaagatttgatcaaagaattttactcacttaaacaaagtcgacctaaacgcgcacagagaaaaactgtaagatctggtccttgggaacctcagtccggcccagcaactctttcatcccccgccaaccaaccacgagaaaaacaaccagcccaacagagaacccccctgctcagctgcccctctcagcccttcacttcaaaactcgccctgcttggacaggtgtttctggactcctcttgatttaaacacgcggccgctaatcagccataccacatttgtagaggttttacttgctttaaaaaacctcccacacctccccctgaacctgaaacataaaatgaatgcaattgttgttgttaacttgtttattgcagcttataatggttacaaataaagcaatagcatcacaaatttcacaaataaagcatttttttcactgcattctagttgtggtttgtccaaactcatcaatgtatcttatcatgtctaccggtagggcccctctcttcatgtgagcaaaaggccagcaaaaggccaggaaccgtaaaaaggccgcgttgctggcgtttttccataggctccgcccccctgacgagcatcacaaaaatcgacgctcaagtcagaggtggcgaaacccgacaggactataaagataccaggcgtttccccctggaagctccctcgtgcgctctcctgttccgaccctgccgcttaccggatacctgtccgcctttctcccttcgggaagcgtggcgctttctcatagctcacgctgtaggtatctcagttcggtgtaggtcgttcgctccaagctgggctgtgtgcacgaaccccccgttcagcccgaccgctgcgccttatccggtaactatcgtcttgagtccaacccggtaagacacgacttatcgccactggcagcagccactggtaacaggattagcagagcgaggtatgtaggcggtgctacagagttcttgaagtggtggcctaactacggctacactagaaggacagtatttggtatctgcgctctgctgaagccagttaccttcggaaaaagagttggtagctcttgatccggcaaacaaaccaccgctggtagcggtggtttttttgtttgcaagcagcagattacgcgcagaaaaaaaggatctcaagaagatcctttgatcttttctacggggtctgacgctcagtggaacgaaaactcacgttaagggattttggtcatgggcgcgcctcatactcctgcaggcatgagattatcaaaaaggatcttcacctagatccttttaaattaaaaatgaagttttaaatcaatctaaagtatatatgagtaaacttggtctgacagttaccaatgcttaatcagtgaggcacctatctcagcgatctgtctatttcgttcatccatagttgcctgactccccgtcgtgtagataactacgatacgggagggcttaccatctggccccagtgctgcaatgataccgcgagacccacgctcaccggctccagatttatcagcaataaaccagccagccggaagggccgagcgcagaagtggtcctgcaactttatccgcctccatccagtctattaattgttgccgggaagctagagtaagtagttcgccagttaatagtttgcgcaacgttgttgccattgctacaggcatcgtggtgtcacgctcgtcgtttggtatggcttcattcagctccggttcccaacgatcaaggcgagttacatgatcccccatgttgtgcaaaaaagcggttagctccttcggtcctccgatcgttgtcagaagtaagttggccgcagtgttatcactcatggttatggcagcactgcataattctcttactgtcatgccatccgtaagatgcttttctgtgactggtgagtactcaaccaagtcattctgagaatagtgtatgcggcgaccgagttgctcttgcccggcgtcaatacgggataataccgcgccacatagcagaactttaaaagtgctcatcattggaaaacgttcttcggggcgaaaactctcaaggatcttaccgctgttgagatccagttcgatgtaacccactcgtgcacccaactgatcttcagcatcttttactttcaccagcgtttctgggtgagcaaaaacaggaaggcaaaatgccgcaaaaaagggaataagggcgacacggaaatgttgaatactcatactcttcctttttcaatattattgaagcatttatcagggttattgtctcatgagcggatacatatttgaatgtatttagaaaaataaacaaataggggttccgcgcacatttccccgaaaagtgccacctgacgtcaggtaccaagcctaggcctccaaaaaagcctcctcactacttctggaatagctcagaggcagaggcggcctcggcctctgcataaataaaaaaaattagtcagccatggggcggagaatgggcggaactgggcggagttaggggcgggatgggcggagttaggggcgggactatggttgctgactaattgagatgcatgctttgcatacttctgcctgctggggagcctggggactttccacacctggttgctgactaattgagatgcatgctttgcatacttctgcctgctggggagcctggggactttccacaccggatccaccatggccaagttgaccagtgccgttccggtgctcaccgcgcgcgacgtcgccggagcggtcgagttctggaccgaccggctcgggttctcccgggacttcgtggaggacgacttcgccggtgtggtccgggacgacgtgaccctgttcatcagcgcggtccaggaccaggtggtgccggacaacaccctggcctgggtgtgggtgcgcggcctggacgagctgtacgccgagtggtcggaggtcgtgtccacgaacttccgggacgcctccgggccggccatgaccgagatcggcgagcagccgtgggggcgggagttcgccctgcgcgacccggccggcaactgcgtgcacttcgtggccgaggagcaggactgaacgcgtgctgtaagtctgcagaaattgatgatctattaaacaataaagatgtccactaaaatggaagtttttcctgtcatactttgttaagaagggtgagaacagagtacctacattttgaatggaaggattggagctacgggggtgggggtggggtgggattagataaatgcctgctctttactgaaggctctttactattgctttatgataatgtttcatagttggatatcataatttaaacaagcaaaaccaaattaagggccagctcattcctcccactcatgatctatggatctatagatctctcgtgcagctggggctctagggggtatccccacgcgccctgtagcggcgcattaagcgcggcgggtgtggtggttacgcgcagcgtgaccgctacacttgccagcgccctagcgcccgctcctttcgctttcttcccttcctttctcgccacgttcgccggctttccccgtcaagctctaaatcgggggctccctttagggttccgatttagtgctttacggcacctcgaccccaaaaaacttgattagggtgatggttcacgtagtgggccatcgccctgatagacggtttttcgccctttgacgttggagtccacgttctttaatagtggactcttgttccaaactggaacaacactcaaccctatctcggtctattcttttgatttataagggattttgccgatttcggcctattggttaaaaaatgagctgatttaacaaaaatttaacgcgaattaattctgtggaatgtgtgtcagttagtcgcgaggcctccgcgccgggttttggcgcctcccgcgggcgcccccctcctcacggcgagcgctgccacgtcagacgaagggcgcagcgagcgtcctgatccttccgcccggacgctcaggacagcggcccgctgctcataagactcggccttagaaccccagtatcagcagaaggacattttaggacgggacttgggtgactctagggcactggttttctttccagagagcggaacaggcgaggaaaagtagtcccttctcggcgattctgcggagggatctccgtggggcggtgaacgccgatgattatataaggacgcgccgggtgtggcacagctagttccgtcgcagccgggatttgggtcgcggttcttgtttgtggatcgctgtgatcgtcacttggtgagtagcgggctgctgggctggccggggctttcgtggccgccgggccgctcggtgggacggaagcgtgtggagagaccgccaagggctgtagtctgggtccgcgagcaaggttgccctgaactgggggttggggggagcgcagcaaaatggcggctgttcccgagtcttgaatggaagacgcttgtgaggcgggctgtgaggtcgttgaaacaaggtggggggcatggtgggcggcaagaacccaaggtcttgaggccttcgctaatgcgggaaagctcttattcgggtgagatgggctggggcaccatctggggaccctgacgtgaagtttgtcactgactggagaactcggtttgtcgtctgttgcgggggcggcagttatggcggtgccgttgggcagtgcacccgtacctttgggagcgcgcgccctcgtcgtgtcgtgacgtcacccgttctgttggcttataatgcagggtggggccacctgccggtaggtgtgcggtaggcttttctccgtcgcaggacgcagggttcgggcctagggtaggctctcctgaatcgacaggcgccggacctctggtgaggggagggataagtgaggcgtcagtttctttggtcggttttatgtacctatcttcttaagtagctgaagctccggttttgaactatgcgctcggggttggcgagtgtgttttgtgaagttttttaggcaccttttgaaatgtaatcatttgggtcaatatgtaattttcagtgttagactagtaaattgtccgctaaattctggccgtttttggcttttttgttagacgtcgaccgatcctgagaacttcagggtgagtttggggacccttgattgttctttctttttcgctattgtaaaattcatgttatatggagggggcaaagttttcagggtgttgtttagaatgggaagatgtcccttgtatcaccatggaccctcatgataattttgtttctttcactttctactctgttgacaaccattgtctcctcttattttcttttcattttctgtaactttttcgttaaactttagcttgcatttgtaacgaatttttaaattcacttttgtttatttgtcagattgtaagtactttctctaatcacttttttttcaaggcaatcagggtatattatattgtacttcagcacagttttagagaacaattgttataattaaatgataaggtagaatatttctgcatataaattctggctggcgtggaaatattcttattggtagaaacaactacaccctggtcatcatcctgcctttctctttatggttacaatgatatacactgtttgagatgaggataaaatactctgagtccaaaccgggcccctctgctaaccatgttcatgccttcttctctttcctacagctcctgggcaacgtgctggttgttgtgctgtctcatcattttggcaaagaatt

SEQ ID NO: 16 - DNA, 3892 bp, Artificial
  Synthetic construct
aggcctccgcgccgggttttggcgcctcccgcgggcgcccccctcctcacggcgagcgctgccacgtcagacgaagggcgcagcgagcgtcctgatccttccgcccggacgctcaggacagcggcccgctgctcataagactcggccttagaaccccagtatcagcagaaggacattttaggacgggacttgggtgactctagggcactggttttctttccagagagcggaacaggcgaggaaaagtagtcccttctcggcgattctgcggagggatctccgtggggcggtgaacgccgatgattatataaggacgcgccgggtgtggcacagctagttccgtcgcagccgggatttgggtcgcggttcttgtttgtggatcgctgtgatcgtcacttggtgagtagcgggctgctgggctggccggggctttcgtggccgccgggccgctcggtgggacggaagcgtgtggagagaccgccaagggctgtagtctgggtccgcgagcaaggttgccctgaactgggggttggggggagcgcagcaaaatggcggctgttcccgagtcttgaatggaagacgcttgtgaggcgggctgtgaggtcgttgaaacaaggtggggggcatggtgggcggcaagaacccaaggtcttgaggccttcgctaatgcgggaaagctcttattcgggtgagatgggctggggcaccatctggggaccctgacgtgaagtttgtcactgactggagaactcggtttgtcgtctgttgcgggggcggcagttatggcggtgccgttgggcagtgcacccgtacctttgggagcgcgcgccctcgtcgtgtcgtgacgtcacccgttctgttggcttataatgcagggtggggccacctgccggtaggtgtgcggtaggcttttctccgtcgcaggacgcagggttcgggcctagggtaggctctcctgaatcgacaggcgccggacctctggtgaggggagggataagtgaggcgtcagtttctttggtcggttttatgtacctatcttcttaagtagctgaagctccggttttgaactatgcgctcggggttggcgagtgtgttttgtgaagttttttaggcaccttttgaaatgtaatcatttgggtcaatatgtaattttcagtgttagactagtaaattgtccgctaaattctggccgtttttggcttttttgttagacgtcgaccgatcctgagaacttcagggtgagtttggggacccttgattgttctttctttttcgctattgtaaaattcatgttatatggagggggcaaagttttcagggtgttgtttagaatgggaagatgtcccttgtatcaccatggaccctcatgataattttgtttctttcactttctactctgttgacaaccattgtctcctcttattttcttttcattttctgtaactttttcgttaaactttagcttgcatttgtaacgaatttttaaattcacttttgtttatttgtcagattgtaagtactttctctaatcacttttttttcaaggcaatcagggtatattatattgtacttcagcacagttttagagaacaattgttataattaaatgataaggtagaatatttctgcatataaattctggctggcgtggaaatattcttattggtagaaacaactacaccctggtcatcatcctgcctttctctttatggttacaatgatatacactgtttgagatgaggataaaatactctgagtccaaaccgggcccctctgctaaccatgttcatgccttcttctctttcctacagctcctgggcaacgtgctggttgttgtgctgtctcatcattttggcaaagaattaagcttatactcgagctctagattgggaacccgggtctctcgaattcgatgccttttagactcctgataccattgggtcttgtttgcgttctcctccctctccatcacggcgccccaggtccagacggtaccgcacctgatcctgcccattaccgcgaacgcgttaaagccatgttctaccacgcctatgactcctatctggaaaatgcattcccctatgatgagctccgaccccttacctgcgatggtcatgatacttggggctctttttcccttacccttattgacgctctggacacactccttatcctcggaaacaccagcgaatttcaaagagtagttgaagtacttcaggacaatgtcgactttgacatcgatgtgaacgcatcagttttcgaaacaaatataagagtcgttggaggtctgctctccgcccaccttctctctaaaaaagccggagtagaagttgaagctggctggccctgctccggacccctccttcgtatggctgaagaagctgcccgcaaactccttcccgcttttcagaccccaaccggtatgccctatggtactgttaacctcctgcacggagtaaatcccggcgaaacccccgtcacatgtacagccggaattggaacctttattgtggaatttgcaacccttagcagcctgaccggagatcctgtattcgaagacgtggctcgggttgccctgatgcgactgtgggaatccaggtctgatatcggtctggtcggtaaccatatagacgtactcactggtaaatgggttgcacaagacgctggaattggggcaggcgtggattcttattttgaatatctcgtaaaaggggccatactcttgcaggacaaaaaacttatggctatgttcctggaatataacaaagctattaggaactacacacacttcgatgattggtatttgtgggtccaaatgtataaaggaaccgtttctatgcctgtctttcagtcactggaggcttattggcctggtctgcaatccctgatcggagacattgacaatgcaatgaggacattccttaattattacactgtttggaagcagttcggcggattgcccgaattttacaacattcctcaaggctatacagttgaaaaaagagaaggatatcccctgcgccccgagcttattgaaagcgctatgtatctgtatcgtgcaacaggtgatccaaccctgcttgaactgggacgagacgccgtcgaatcaatcgagaaaatttcaaaagtggaatgcggctttgcaacaattaaagatcttagagaccacaaactggataatcgcatggagtcattctttttggctgagaccgtcaagtatctgtatctgctttttcatcccaacaacttcatccataataacgggtccaccttcgattcagtcatgacccctcacggtgaatgcatactcggagctggaggctatatttttaacactgaagctcacccaattgacccagctgcccttcattgttgtcgacgtctgaaagaagaacaatgggaggttgaagatttgatcaaagaattttactcacttaaacaaagtcgacctaaacgcgcacagagaaaaactgtaagatctggtccttgggaacctcagtccggcccagcaactctttcatcccccgccaaccaaccacgagaaaaacaaccagcccaacagagaacccccctgctcagctgcccctctcagcccttcacttcaaaactcgccctgcttggacaggtgtttctggactcctcttgatttaaacacgcggccgctaatcagccataccacatttgtagaggttttacttgctttaaaaaacctcccacacctccccctgaacctgaaacataaaatgaatgcaattgttgttgttaacttgtttattgcagcttataatggttacaaataaagcaatagcatcacaaatttcacaaataaagcatttttttcactgcattctagttgtggtttgtccaaactcatcaatgtatcttatcatgt

SEQ ID NO: 17 - DNA, 6629 bp, Artificial
  Synthetic plasmid
aagcttatactcgagctctagattgggaacccgggtctctcgaattcatggtggtggtggctgctgctccttctgctgctacagctgctcctaaggtgctgctgctgtctggacagcctgcttctggaggaagagctctgcctctgatggtgcctggacctagagctgctggatctgaggcttctggaacacctcaggctagaaagagacagagactgacacatctgtctcctgaagaaaaggctctgagaagaaagctgaagaatagagtggctgctcagacagctagagatagaaagaaggctagaatgtctgaactggaacagcaggtggtggatctggaagaagaaaatcataagctgcagctggaaaatcagctgctgagagaaaagacacatggactggtggtggaaaatcaggaactgagaacaagactgggaatggatacactggatcctgatgaagtgcctgaagtggaagctaagggatctggagtgagactggtggctggatctgctgaatctgctgctggagctggacctgtggtgacatctcctgaacatctgcctatggattctgatacagtggcttcttctgattctgaatctgatatcctgctgggaatcctggataagctggatcctgtgatgttttttaagtgtccttctcctgaatctgcttctctggaagaactgcctgaagtgtatcctgaaggaccttcttctctgcctgcttctctgtctctgtctgtgggaacatcttctgctaagctggaagctatcaatgaactgatcagatttgatcatgtgtatacaaagcctctggtgctggaaatcccttctgaaacagaatctcagacaaatgtggtggtgaagatcgaagaagctcctctgtcttcttctgaagaagatcatcctgaatttatcgtgtctgtgaagaaggaacctctggaagatgattttatccctgaactgggaatctctaatctgctgtcttcttctcattgtctgagacctccttcttgtctgctggatgctcattctgattgtggatatgaaggatctccttctcctttttctgatatgtcttctcctctgggaacagatcattcttgggaagatacatttgctaatgaactgtttcctcagctgatctctgtgtgagcggccgctaatcagccataccacatttgtagaggttttacttgctttaaaaaacctcccacacctccccctgaacctgaaacataaaatgaatgcaattgttgttgttaacttgtttattgcagcttataatggttacaaataaagcaatagcatcacaaatttcacaaataaagcatttttttcactgcattctagttgtggtttgtccaaactcatcaatgtatcttatcatgtctaccggtagggcccctctcttcatgtgagcaaaaggccagcaaaaggccaggaaccgtaaaaaggccgcgttgctggcgtttttccataggctccgcccccctgacgagcatcacaaaaatcgacgctcaagtcagaggtggcgaaacccgacaggactataaagataccaggcgtttccccctggaagctccctcgtgcgctctcctgttccgaccctgccgcttaccggatacctgtccgcctttctcccttcgggaagcgtggcgctttctcatagctcacgctgtaggtatctcagttcggtgtaggtcgttcgctccaagctgggctgtgtgcacgaaccccccgttcagcccgaccgctgcgccttatccggtaactatcgtcttgagtccaacccggtaagacacgacttatcgccactggcagcagccactggtaacaggattagcagagcgaggtatgtaggcggtgctacagagttcttgaagtggtggcctaactacggctacactagaaggacagtatttggtatctgcgctctgctgaagccagttaccttcggaaaaagagttggtagctcttgatccggcaaacaaaccaccgctggtagcggtggtttttttgtttgcaagcagcagattacgcgcagaaaaaaaggatctcaagaagatcctttgatcttttctacggggtctgacgctcagtggaacgaaaactcacgttaagggattttggtcatgggcgcgcctcatactcctgcaggcatgagattatcaaaaaggatcttcacctagatccttttaaattaaaaatgaagttttaaatcaatctaaagtatatatgagtaaacttggtctgacagttaccaatgcttaatcagtgaggcacctatctcagcgatctgtctatttcgttcatccatagttgcctgactccccgtcgtgtagataactacgatacgggagggcttaccatctggccccagtgctgcaatgataccgcgagacccacgctcaccggctccagatttatcagcaataaaccagccagccggaagggccgagcgcagaagtggtcctgcaactttatccgcctccatccagtctattaattgttgccgggaagctagagtaagtagttcgccagttaatagtttgcgcaacgttgttgccattgctacaggcatcgtggtgtcacgctcgtcgtttggtatggcttcattcagctccggttcccaacgatcaaggcgagttacatgatcccccatgttgtgcaaaaaagcggttagctccttcggtcctccgatcgttgtcagaagtaagttggccgcagtgttatcactcatggttatggcagcactgcataattctcttactgtcatgccatccgtaagatgcttttctgtgactggtgagtactcaaccaagtcattctgagaatagtgtatgcggcgaccgagttgctcttgcccggcgtcaatacgggataataccgcgccacatagcagaactttaaaagtgctcatcattggaaaacgttcttcggggcgaaaactctcaaggatcttaccgctgttgagatccagttcgatgtaacccactcgtgcacccaactgatcttcagcatcttttactttcaccagcgtttctgggtgagcaaaaacaggaaggcaaaatgccgcaaaaaagggaataagggcgacacggaaatgttgaatactcatactcttcctttttcaatattattgaagcatttatcagggttattgtctcatgagcggatacatatttgaatgtatttagaaaaataaacaaataggggttccgcgcacatttccccgaaaagtgccacctgacgtcaggtaccaagcctaggcctccaaaaaagcctcctcactacttctggaatagctcagaggcagaggcggcctcggcctctgcataaataaaaaaaattagtcagccatggggcggagaatgggcggaactgggcggagttaggggcgggatgggcggagttaggggcgggactatggttgctgactaattgagatgcatgctttgcatacttctgcctgctggggagcctggggactttccacacctggttgctgactaattgagatgcatgctttgcatacttctgcctgctggggagcctggggactttccacaccggatccaccatggccaagttgaccagtgccgttccggtgctcaccgcgcgcgacgtcgccggagcggtcgagttctggaccgaccggctcgggttctcccgggacttcgtggaggacgacttcgccggtgtggtccgggacgacgtgaccctgttcatcagcgcggtccaggaccaggtggtgccggacaacaccctggcctgggtgtgggtgcgcggcctggacgagctgtacgccgagtggtcggaggtcgtgtccacgaacttccgggacgcctccgggccggccatgaccgagatcggcgagcagccgtgggggcgggagttcgccctgcgcgacccggccggcaactgcgtgcacttcgtggccgaggagcaggactgaacgcgtgctgtaagtctgcagaaattgatgatctattaaacaataaagatgtccactaaaatggaagtttttcctgtcatactttgttaagaagggtgagaacagagtacctacattttgaatggaaggattggagctacgggggtgggggtggggtgggattagataaatgcctgctctttactgaaggctctttactattgctttatgataatgtttcatagttggatatcataatttaaacaagcaaaaccaaattaagggccagctcattcctcccactcatgatctatggatctatagatctctcgtgcagctggggctctagggggtatccccacgcgccctgtagcggcgcattaagcgcggcgggtgtggtggttacgcgcagcgtgaccgctacacttgccagcgccctagcgcccgctcctttcgctttcttcccttcctttctcgccacgttcgccggctttccccgtcaagctctaaatcgggggctccctttagggttccgatttagtgctttacggcacctcgaccccaaaaaacttgattagggtgatggttcacgtagtgggccatcgccctgatagacggtttttcgccctttgacgttggagtccacgttctttaatagtggactcttgttccaaactggaacaacactcaaccctatctcggtctattcttttgatttataagggattttgccgatttcggcctattggttaaaaaatgagctgatttaacaaaaatttaacgcgaattaattctgtggaatgtgtgtcagttagtcgcgaggcctccgcgccgggttttggcgcctcccgcgggcgcccccctcctcacggcgagcgctgccacgtcagacgaagggcgcagcgagcgtcctgatccttccgcccggacgctcaggacagcggcccgctgctcataagactcggccttagaaccccagtatcagcagaaggacattttaggacgggacttgggtgactctagggcactggttttctttccagagagcggaacaggcgaggaaaagtagtcccttctcggcgattctgcggagggatctccgtggggcggtgaacgccgatgattatataaggacgcgccgggtgtggcacagctagttccgtcgcagccgggatttgggtcgcggttcttgtttgtggatcgctgtgatcgtcacttggtgagtagcgggctgctgggctggccggggctttcgtggccgccgggccgctcggtgggacggaagcgtgtggagagaccgccaagggctgtagtctgggtccgcgagcaaggttgccctgaactgggggttggggggagcgcagcaaaatggcggctgttcccgagtcttgaatggaagacgcttgtgaggcgggctgtgaggtcgttgaaacaaggtggggggcatggtgggcggcaagaacccaaggtcttgaggccttcgctaatgcgggaaagctcttattcgggtgagatgggctggggcaccatctggggaccctgacgtgaagtttgtcactgactggagaactcggtttgtcgtctgttgcgggggcggcagttatggcggtgccgttgggcagtgcacccgtacctttgggagcgcgcgccctcgtcgtgtcgtgacgtcacccgttctgttggcttataatgcagggtggggccacctgccggtaggtgtgcggtaggcttttctccgtcgcaggacgcagggttcgggcctagggtaggctctcctgaatcgacaggcgccggacctctggtgaggggagggataagtgaggcgtcagtttctttggtcggttttatgtacctatcttcttaagtagctgaagctccggttttgaactatgcgctcggggttggcgagtgtgttttgtgaagttttttaggcaccttttgaaatgtaatcatttgggtcaatatgtaattttcagtgttagactagtaaattgtccgctaaattctggccgtttttggcttttttgttagacgtcgaccgatcctgagaacttcagggtgagtttggggacccttgattgttctttctttttcgctattgtaaaattcatgttatatggagggggcaaagttttcagggtgttgtttagaatgggaagatgtcccttgtatcaccatggaccctcatgataattttgtttctttcactttctactctgttgacaaccattgtctcctcttattttcttttcattttctgtaactttttcgttaaactttagcttgcatttgtaacgaatttttaaattcacttttgtttatttgtcagattgtaagtactttctctaatcacttttttttcaaggcaatcagggtatattatattgtacttcagcacagttttagagaacaattgttataattaaatgataaggtagaatatttctgcatataaattctggctggcgtggaaatattcttattggtagaaacaactacaccctggtcatcatcctgcctttctctttatggttacaatgatatacactgtttgagatgaggataaaatactctgagtccaaaccgggcccctctgctaaccatgttcatgccttcttctctttcctacagctcctgggcaacgtgctggttgttgtgctgtctcatcattttggcaaagaatt

SEQ ID NO: 18 - DNA, 3264 bp, Artificial
  Synthetic construct
ggcctccgcgccgggttttggcgcctcccgcgggcgcccccctcctcacggcgagcgctgccacgtcagacgaagggcgcagcgagcgtcctgatccttccgcccggacgctcaggacagcggcccgctgctcataagactcggccttagaaccccagtatcagcagaaggacattttaggacgggacttgggtgactctagggcactggttttctttccagagagcggaacaggcgaggaaaagtagtcccttctcggcgattctgcggagggatctccgtggggcggtgaacgccgatgattatataaggacgcgccgggtgtggcacagctagttccgtcgcagccgggatttgggtcgcggttcttgtttgtggatcgctgtgatcgtcacttggtgagtagcgggctgctgggctggccggggctttcgtggccgccgggccgctcggtgggacggaagcgtgtggagagaccgccaagggctgtagtctgggtccgcgagcaaggttgccctgaactgggggttggggggagcgcagcaaaatggcggctgttcccgagtcttgaatggaagacgcttgtgaggcgggctgtgaggtcgttgaaacaaggtggggggcatggtgggcggcaagaacccaaggtcttgaggccttcgctaatgcgggaaagctcttattcgggtgagatgggctggggcaccatctggggaccctgacgtgaagtttgtcactgactggagaactcggtttgtcgtctgttgcgggggcggcagttatggcggtgccgttgggcagtgcacccgtacctttgggagcgcgcgccctcgtcgtgtcgtgacgtcacccgttctgttggcttataatgcagggtggggccacctgccggtaggtgtgcggtaggcttttctccgtcgcaggacgcagggttcgggcctagggtaggctctcctgaatcgacaggcgccggacctctggtgaggggagggataagtgaggcgtcagtttctttggtcggttttatgtacctatcttcttaagtagctgaagctccggttttgaactatgcgctcggggttggcgagtgtgttttgtgaagttttttaggcaccttttgaaatgtaatcatttgggtcaatatgtaattttcagtgttagactagtaaattgtccgctaaattctggccgtttttggcttttttgttagacgtcgaccgatcctgagaacttcagggtgagtttggggacccttgattgttctttctttttcgctattgtaaaattcatgttatatggagggggcaaagttttcagggtgttgtttagaatgggaagatgtcccttgtatcaccatggaccctcatgataattttgtttctttcactttctactctgttgacaaccattgtctcctcttattttcttttcattttctgtaactttttcgttaaactttagcttgcatttgtaacgaatttttaaattcacttttgtttatttgtcagattgtaagtactttctctaatcacttttttttcaaggcaatcagggtatattatattgtacttcagcacagttttagagaacaattgttataattaaatgataaggtagaatatttctgcatataaattctggctggcgtggaaatattcttattggtagaaacaactacaccctggtcatcatcctgcctttctctttatggttacaatgatatacactgtttgagatgaggataaaatactctgagtccaaaccgggcccctctgctaaccatgttcatgccttcttctctttcctacagctcctgggcaacgtgctggttgttgtgctgtctcatcattttggcaaagaattaagcttatactcgagctctagattgggaacccgggtctctcgaattcatggtggtggtggctgctgctccttctgctgctacagctgctcctaaggtgctgctgctgtctggacagcctgcttctggaggaagagctctgcctctgatggtgcctggacctagagctgctggatctgaggcttctggaacacctcaggctagaaagagacagagactgacacatctgtctcctgaagaaaaggctctgagaagaaagctgaagaatagagtggctgctcagacagctagagatagaaagaaggctagaatgtctgaactggaacagcaggtggtggatctggaagaagaaaatcataagctgcagctggaaaatcagctgctgagagaaaagacacatggactggtggtggaaaatcaggaactgagaacaagactgggaatggatacactggatcctgatgaagtgcctgaagtggaagctaagggatctggagtgagactggtggctggatctgctgaatctgctgctggagctggacctgtggtgacatctcctgaacatctgcctatggattctgatacagtggcttcttctgattctgaatctgatatcctgctgggaatcctggataagctggatcctgtgatgttttttaagtgtccttctcctgaatctgcttctctggaagaactgcctgaagtgtatcctgaaggaccttcttctctgcctgcttctctgtctctgtctgtgggaacatcttctgctaagctggaagctatcaatgaactgatcagatttgatcatgtgtatacaaagcctctggtgctggaaatcccttctgaaacagaatctcagacaaatgtggtggtgaagatcgaagaagctcctctgtcttcttctgaagaagatcatcctgaatttatcgtgtctgtgaagaaggaacctctggaagatgattttatccctgaactgggaatctctaatctgctgtcttcttctcattgtctgagacctccttcttgtctgctggatgctcattctgattgtggatatgaaggatctccttctcctttttctgatatgtcttctcctctgggaacagatcattcttgggaagatacatttgctaatgaactgtttcctcagctgatctctgtgtgagcggccgctaatcagccataccacatttgtagaggttttacttgctttaaaaaacctcccacacctccccctgaacctgaaacataaaatgaatgcaattgttgttgttaacttgtttattgcagcttataatggttacaaataaagcaatagcatcacaaatttcacaaataaagcatttttttcactgcattctagttgtggtttgtccaaactcatcaatgtatcttatcatgtc

SEQ ID NO: 19 - protein, 447 aa, Homo sapiens
EVQVLESGGDLVQPGGSLRLSCAASGFTFSAYAMTWVRQAPGKGLEWVSAISGSGGSAYYADSVKGRFTISRDNSKNTVYLQMNSLRAEDTAVYYCAKDGAWKMSGLDVWGQGTTVIVSSASTKGPSVFPLAPCSRSTSESTAALGCLVKDYFPEPVTVSWNSGALTSGVHTFPAVLQSSGLYSLSSVVTVPSSSLGTKTYTCNVDHKPSNTKVDKRVESKYGPPCPPCPAPEFLGGPSVFLFPPKPKDTLMISRTPEVTCVVVDVSQEDPEVQFNWYVDGVEVHNAKTKPREEQFNSTYRVVSVLTVLHQDWLNGKEYKCKVSNKGLPSSIEKTISKAKGQPREPQVYTLPPSQEEMTKNQVSLTCLVKGFYPSDIAVEWESNGQPENNYKTTPPVLDSDGSFFLYSRLTVDKSRWQEGNVFSCSVMHEALHNHYTQKSLSLSLGK

SEQ ID NO: 20 - protein, 110 aa, Homo sapiens
ESGGDLVQPGGSLRLSCAASGFTFSAYAMTWVRQAPGKGLEWVSAISGSGGSAYYADSVKGRFTISRDNSKNTVYLQMNSLRAEDTAVYYCAKDGAWKMSGLDVWGQGTT

SEQ ID NO: 21 - protein, 214 aa, Homo sapiens
DIQMTQSPASLSASVGDRVTITCRASQDISDYLAWYQQKPGKIPRLLIYTTSTLQSGVPSRFRGSGSGTDFTLTISSLQPEDVATYYCQKYDSAPLTFGGGTKVEIKRTVAAPSVFIFPPSDEQLKSGTASVVCLLNNFYPREAKVQWKVDNALQSGNSQESVTEQDSKDSTYSLSSTLTLSKADYEKHKVYACEVTHQGLSSPVTKSFNRGEC

SEQ ID NO: 22 - protein, 100 aa, Homo sapiens
QSPASLSASVGDRVTITCRASQDISDYLAWYQQKPGKIPRLLIYTTSTLQSGVPSRFRGSGSGTDFTLTISSLQPEDVATYYCQKYDSAPLTFGGGTKVE

SEQ ID NO: 23 - DNA, 2971 bp, Artificial
  Synthetic construct
tagttattaatagtaatcaattacggggtcattagttcatagcccatatatggagttccgcgttacataacttacggtaaatggcccgcctggctgaccgcccaacgacccccgcccattgacgtcaataatgacgtatgttcccatagtaacgccaatagggactttccattgacgtcaatgggtggagtatttacggtaaactgcccacttggcagtacatcaagtgtatcatatgccaagtacgccccctattgacgtcaatgacggtaaatggcccgcctggcattatgcccagtacatgaccttatgggactttcctacttggcagtacatctacgtattagtcatcgctattaccatggtgatgcggttttggcagtacatcaatgggcgtggatagcggtttgactcacggggatttccaagtctccaccccattgacgtcaatgggagtttgttttggcaccaaaatcaacgggactttccaaaatgtcgtaacaactccgccccattgacgcaaatgggcggtaggcgtgtacggtgggaggtctatataagcagagctcatgatagaagcactctactattcgtcgaccgatcctgagaacttcagggtgagtttggggacccttgattgttctttctttttcgctattgtaaaattcatgttatatggagggggcaaagttttcagggtgttgtttagaatgggaagatgtcccttgtatcaccatggaccctcatgataattttgtttctttcactttctactctgttgacaaccattgtctcctcttattttcttttcattttctgtaactttttcgttaaactttagcttgcatttgtaacgaatttttaaattcacttttgtttatttgtcagattgtaagtactttctctaatcacttttttttcaaggcaatcagggtatattatattgtacttcagcacagttttagagaacaattgttataattaaatgataaggtagaatatttctgcatataaattctggctggcgtggaaatattcttattggtagaaacaactacaccctggtcatcatcctgcctttctctttatggttacaatgatatacactgtttgagatgaggataaaatactctgagtccaaaccgggcccctctgctaaccatgttcatgccttcttctctttcctacagctcctgggcaacgtgctggttgttgtgctgtctcatcattttggcaaagaattaagcttatactcgagctctagattgggaacccgggtctctcgaattcgagatctccaccatgcacagacctagacgtcgtggaactcgtccacctccactggcactgctcgctgctctcctcctggctgcacgtggtgctgatgcagaggtgcaggtgttggagtctgggggagacttggtacagcctggggggtccctgagactctcctgtgcagcctctggattcacctttagtgcctatgccatgacctgggtccgccaggctccagggaaggggctggagtgggtctcagctattagtggtagtggtggtagcgcatactacgcagactccgtgaagggccggttcaccatctccagagacaattccaagaacacggtatatctgcagatgaacagcctgagagccgaggacacggccgtatattactgtgcgaaagatggggcctggaaaatgtccggtttggacgtctggggccaagggaccacggtcatcgtctcctcagcctccaccaagggcccatcggtcttccccctggcgccctgctccaggagcacctccgagagcacagccgccctgggctgcctggtcaaggactacttccccgaaccggtgacggtgtcgtggaactcaggcgccctgaccagcggcgtgcacaccttcccggctgtcctacagtcctcaggactctactccctcagcagcgtggtgaccgtgccctccagcagcttgggcacgaagacctacacctgcaacgtagatcacaagcccagcaacaccaaggtggacaagagagttgagtccaaatatggtcccccatgcccaccctgcccagcacctgagttcctggggggaccatcagtcttcctgttccccccaaaacccaaggacactctcatgatctcccggacccctgaggtcacgtgcgtggtggtggacgtgagccaggaagaccccgaggtccagttcaactggtacgtggatggcgtggaggtgcataatgccaagacaaagccgcgggaggagcagttcaacagcacgtaccgtgtggtcagcgtcctcaccgtcctgcaccaggactggctgaacggcaaggagtacaagtgcaaggtctccaacaaaggcctcccgtcctccatcgagaaaaccatctccaaagccaaagggcagccccgagagccacaggtgtacaccctgcccccatcccaggaggagatgaccaagaaccaggtcagcctgacctgcctggtcaaaggcttctaccccagcgacatcgccgtggagtgggagagcaatgggcagccggagaacaactacaagaccacgcctcccgtgctggactccgacggctccttcttcctctacagcaggctcaccgtggacaagagcaggtggcaggaggggaatgtcttctcatgctccgtgatgcatgaggctctgcacaaccactacacacagaagtccctctccctgtctctgggtaaatgagcggccgctaatcagccataccacatttgtagaggttttacttgctttaaaaaacctcccacacctccccctgaacctgaaacataaaatgaatgcaattgttgttgttaacttgtttattgcagcttataatggttacaaataaagcaatagcatcacaaatttcacaaataaagcatttttttcactgcattctagttgtggtttgtccaaactcatcaatgtatcttatcatgtc

SEQ ID NO: 24 - DNA, 7013 bp, Artificial
  Synthetic plasmid
tcgcgatgtgtgactagttagttattaatagtaatcaattacggggtcattagttcatagcccatatatggagttccgcgttacataacttacggtaaatggcccgcctggctgaccgcccaacgacccccgcccattgacgtcaataatgacgtatgttcccatagtaacgccaatagggactttccattgacgtcaatgggtggagtatttacggtaaactgcccacttggcagtacatcaagtgtatcatatgccaagtacgccccctattgacgtcaatgacggtaaatggcccgcctggcattatgcccagtacatgaccttatgggactttcctacttggcagtacatctacgtattagtcatcgctattaccatggtgatgcggttttggcagtacatcaatgggcgtggatagcggtttgactcacggggatttccaagtctccaccccattgacgtcaatgggagtttgttttggcaccaaaatcaacgggactttccaaaatgtcgtaacaactccgccccattgacgcaaatgggcggtaggcgtgtacggtgggaggtctatataagcagagctcatgatagaagcactctactattcgtcgaccgatcctgagaacttcagggtgagtttggggacccttgattgttctttctttttcgctattgtaaaattcatgttatatggagggggcaaagttttcagggtgttgtttagaatgggaagatgtcccttgtatcaccatggaccctcatgataattttgtttctttcactttctactctgttgacaaccattgtctcctcttattttcttttcattttctgtaactttttcgttaaactttagcttgcatttgtaacgaatttttaaattcacttttgtttatttgtcagattgtaagtactttctctaatcacttttttttcaaggcaatcagggtatattatattgtacttcagcacagttttagagaacaattgttataattaaatgataaggtagaatatttctgcatataaattctggctggcgtggaaatattcttattggtagaaacaactacaccctggtcatcatcctgcctttctctttatggttacaatgatatacactgtttgagatgaggataaaatactctgagtccaaaccgggcccctctgctaaccatgttcatgccttcttctctttcctacagctcctgggcaacgtgctggttgttgtgctgtctcatcattttggcaaagaattaagcttatactcgagctctagattgggaacccgggtctctcgaattcgagatctccaccatgcacagacctagacgtcgtggaactcgtccacctccactggcactgctcgctgctctcctcctggctgcacgtggtgctgatgcagaggtgcaggtgttggagtctgggggagacttggtacagcctggggggtccctgagactctcctgtgcagcctctggattcacctttagtgcctatgccatgacctgggtccgccaggctccagggaaggggctggagtgggtctcagctattagtggtagtggtggtagcgcatactacgcagactccgtgaagggccggttcaccatctccagagacaattccaagaacacggtatatctgcagatgaacagcctgagagccgaggacacggccgtatattactgtgcgaaagatggggcctggaaaatgtccggtttggacgtctggggccaagggaccacggtcatcgtctcctcagcctccaccaagggcccatcggtcttccccctggcgccctgctccaggagcacctccgagagcacagccgccctgggctgcctggtcaaggactacttccccgaaccggtgacggtgtcgtggaactcaggcgccctgaccagcggcgtgcacaccttcccggctgtcctacagtcctcaggactctactccctcagcagcgtggtgaccgtgccctccagcagcttgggcacgaagacctacacctgcaacgtagatcacaagcccagcaacaccaaggtggacaagagagttgagtccaaatatggtcccccatgcccaccctgcccagcacctgagttcctggggggaccatcagtcttcctgttccccccaaaacccaaggacactctcatgatctcccggacccctgaggtcacgtgcgtggtggtggacgtgagccaggaagaccccgaggtccagttcaactggtacgtggatggcgtggaggtgcataatgccaagacaaagccgcgggaggagcagttcaacagcacgtaccgtgtggtcagcgtcctcaccgtcctgcaccaggactggctgaacggcaaggagtacaagtgcaaggtctccaacaaaggcctcccgtcctccatcgagaaaaccatctccaaagccaaagggcagccccgagagccacaggtgtacaccctgcccccatcccaggaggagatgaccaagaaccaggtcagcctgacctgcctggtcaaaggcttctaccccagcgacatcgccgtggagtgggagagcaatgggcagccggagaacaactacaagaccacgcctcccgtgctggactccgacggctccttcttcctctacagcaggctcaccgtggacaagagcaggtggcaggaggggaatgtcttctcatgctccgtgatgcatgaggctctgcacaaccactacacacagaagtccctctccctgtctctgggtaaatgagcggccgctaatcagccataccacatttgtagaggttttacttgctttaaaaaacctcccacacctccccctgaacctgaaacataaaatgaatgcaattgttgttgttaacttgtttattgcagcttataatggttacaaataaagcaatagcatcacaaatttcacaaataaagcatttttttcactgcattctagttgtggtttgtccaaactcatcaatgtatcttatcatgtctaccggtcctgcagggcccctctcttcatgtgagcaaaaggccagcaaaaggccaggaaccgtaaaaaggccgcgttgctggcgtttttccataggctccgcccccctgacgagcatcacaaaaatcgacgctcaagtcagaggtggcgaaacccgacaggactataaagataccaggcgtttccccctggaagctccctcgtgcgctctcctgttccgaccctgccgcttaccggatacctgtccgcctttctcccttcgggaagcgtggcgctttctcaatgctcacgctgtaggtatctcagttcggtgtaggtcgttcgctccaagctgggctgtgtgcacgaaccccccgttcagcccgaccgctgcgccttatccggtaactatcgtcttgagtccaacccggtaagacacgacttatcgccactggcagcagccactggtaacaggattagcagagcgaggtatgtaggcggtgctacagagttcttgaagtggtggcctaactacggctacactagaaggacagtatttggtatctgcgctctgctgaagccagttaccttcggaaaaagagttggtagctcttgatccggcaaacaaaccaccgctggtagcggtggtttttttgtttgcaagcagcagattacgcgcagaaaaaaaggatctcaagaagatcctttgatcttttctacggggtctgacgctcagtggaacgaaaactcacgttaagggattttggtcatgggcgcgcctcatactcctgcaggcatgagattatcaaaaaggatcttcacctagatccttttaaattaaaaatgaagttttaaatcaatctaaagtatatatgagtaaacttggtctgacagttaccaatgcttaatcagtgaggcacctatctcagcgatctgtctatttcgttcatccatagttgcctgactccccgtcgtgtagataactacgatacgggagggcttaccatctggccccagtgctgcaatgataccgcgagacccacgctcaccggctccagatttatcagcaataaaccagccagccggaagggccgagcgcagaagtggtcctgcaactttatccgcctccatccagtctattaattgttgccgggaagctagagtaagtagttcgccagttaatagtttgcgcaacgttgttgccattgctacaggcatcgtggtgtcacgctcgtcgtttggtatggcttcattcagctccggttcccaacgatcaaggcgagttacatgatcccccatgttgtgcaaaaaagcggttagctccttcggtcctccgatcgttgtcagaagtaagttggccgcagtgttatcactcatggttatggcagcactgcataattctcttactgtcatgccatccgtaagatgcttttctgtgactggtgagtactcaaccaagtcattctgagaatagtgtatgcggcgaccgagttgctcttgcccggcgtcaatacgggataataccgcgccacatagcagaactttaaaagtgctcatcattggaaaacgttcttcggggcgaaaactctcaaggatcttaccgctgttgagatccagttcgatgtaacccactcgtgcacccaactgatcttcagcatcttttactttcaccagcgtttctgggtgagcaaaaacaggaaggcaaaatgccgcaaaaaagggaataagggcgacacggaaatgttgaatactcatactcttcctttttcaatattattgaagcatttatcagggttattgtctcatgagcggatacatatttgaatgtatttagaaaaataaacaaataggggttccgcgcacatttccccgaaaagtgccacctgacgtcaggtaccaagcctaggcctccaaaaaagcctcctcactacttctggaatagctcagaggcagaggcggcctcggcctctgcataaataaaaaaaattagtcagccatggggcggagaatgggcggaactgggcggagttaggggcgggatgggcggagttaggggcgggactatggttgctgactaattgagatgcatgctttgcatacttctgcctgctggggagcctggggactttccacacctggttgctgactaattgagatgcatgctttgcatacttctgcctgctggggagcctggggactttccacaccggatccaccatggatagatccggaaagcctgaactcaccgcgacgtctgtcgagaagtttctgatcgaaaagttcgacagcgtctccgacctgatgcagctctcggagggcgaagaatctcgtgctttcagcttcgatgtaggagggcgtggatatgtcctgcgggtaaatagctgcgccgatggtttctacaaagatcgttatgtttatcggcactttgcatcggccgcgctcccgattccggaagtgcttgacattggggagttcagcgagagcctgacctattgcatctcccgccgtgcacagggtgtcacgttgcaagacctgcctgaaaccgaactgcccgctgttctgcagccggtcgcggaggccatggatgcgatcgctgcggccgatcttagccagacgagcgggttcggcccattcggaccgcaaggaatcggtcaatacactacatggcgtgatttcatatgcgcgattgctgatccccatgtgtatcactggcaaactgtgatggacgacaccgtcagtgcgtccgtcgcgcaggctctcgatgagctgatgctttgggccgaggactgccccgaagtccggcacctcgtgcacgcggatttcggctccaacaatgtcctgacggacaatggccgcataacagcggtcattgactggagcgaggcgatgttcggggattcccaatacgaggtcgccaacatcttcttctggaggccgtggttggcttgtatggagcagcagacgcgctacttcgagcggaggcatccggagcttgcaggatcgccgcggctccgggcgtatatgctccgcattggtcttgaccaactctatcagagcttggttgacggcaatttcgatgatgcagcttgggcgcagggtcgatgcgacgcaatcgtccgatccggagccgggactgtcgggcgtacacaaatcgcccgcagaagcgcggccgtctggaccgatggctgtgtagaagtactcgccgatagtggaaaccgacgccccagcactcgtccgagggcaaaggaatagacgcgtgctgtaagtctgcagaaattgatgatctattaaacaataaagatgtccactaaaatggaagtttttcctgtcatactttgttaagaagggtgagaacagagtacctacattttgaatggaaggattggagctacgggggtgggggtggggtgggattagataaatgcctgctctttactgaaggctctttactattgctttatgataatgtttcatagttggatatcataatttaaacaagcaaaaccaaattaagggccagctcattcctcccactcatgatctatggatctatagatctctcgtgcagctggggctctagggggtatccccacgcgccctgtagcggcgcattaagcgcggcgggtgtggtggttacgcgcagcgtgaccgctacacttgccagcgccctagcgcccgctcctttcgctttcttcccttcctttctcgccacgttcgccggctttccccgtcaagctctaaatcgggggctccctttagggttccgatttagtgctttacggcacctcgaccccaaaaaacttgattagggtgatggttcacgtagtgggccatcgccctgatagacggtttttcgccctttgacgttggagtccacgttctttaatagtggactcttgttccaaactggaacaacactcaaccctatctcggtctattcttttgatttataagggattttgccgatttcggcctattggttaaaaaatgagctgatttaacaaaaatttaacgcgaattaattctgtggaatgtgtgtcagttag

SEQ ID NO: 25 - DNA, 2272 bp, Artificial
  Synthetic construct
tagttattaatagtaatcaattacggggtcattagttcatagcccatatatggagttccgcgttacataacttacggtaaatggcccgcctggctgaccgcccaacgacccccgcccattgacgtcaataatgacgtatgttcccatagtaacgccaatagggactttccattgacgtcaatgggtggagtatttacggtaaactgcccacttggcagtacatcaagtgtatcatatgccaagtacgccccctattgacgtcaatgacggtaaatggcccgcctggcattatgcccagtacatgaccttatgggactttcctacttggcagtacatctacgtattagtcatcgctattaccatggtgatgcggttttggcagtacatcaatgggcgtggatagcggtttgactcacggggatttccaagtctccaccccattgacgtcaatgggagtttgttttggcaccaaaatcaacgggactttccaaaatgtcgtaacaactccgccccattgacgcaaatgggcggtaggcgtgtacggtgggaggtctatataagcagagctcatgatagaagcactctactattcgtcgaccgatcctgagaacttcagggtgagtttggggacccttgattgttctttctttttcgctattgtaaaattcatgttatatggagggggcaaagttttcagggtgttgtttagaatgggaagatgtcccttgtatcaccatggaccctcatgataattttgtttctttcactttctactctgttgacaaccattgtctcctcttattttcttttcattttctgtaactttttcgttaaactttagcttgcatttgtaacgaatttttaaattcacttttgtttatttgtcagattgtaagtactttctctaatcacttttttttcaaggcaatcagggtatattatattgtacttcagcacagttttagagaacaattgttataattaaatgataaggtagaatatttctgcatataaattctggctggcgtggaaatattcttattggtagaaacaactacaccctggtcatcatcctgcctttctctttatggttacaatgatatacactgtttgagatgaggataaaatactctgagtccaaaccgggcccctctgctaaccatgttcatgccttcttctctttcctacagctcctgggcaacgtgctggttgttgtgctgtctcatcattttggcaaagaattaagcttatactcgagctctagattgggaacccgggtctctcgaattcgagatctccaccatgcacagacctagacgtcgtggaactcgtccacctccactggcactgctcgctgctctcctcctggctgcacgtggtgctgatgcagacatccagatgacccagtctccagcctccctgtctgcatctgttggagacagagtcaccatcacttgtcgggcgagtcaggacattagcgattatttagcctggtatcagcagaaaccagggaaaattcctaggctcctgatctatactacatccactttgcaatcaggggtcccatctcggttccgtggcagtgggtctgggacagatttcactctcaccatcagcagcctgcagcctgaagatgttgcaacttattactgtcagaagtatgacagtgccccgctcactttcggcggagggaccaaggtggagatcaaacgaactgtggctgcaccatctgtcttcatcttcccgccatctgatgagcagttgaaatctggaactgcctctgttgtgtgcctgctgaataacttctatcccagagaggccaaagtacagtggaaggtggataacgccctccaatcgggtaactcccaggagagtgtcacagagcaggacagcaaggacagcacctacagcctcagcagcaccctgacgctgagcaaagcagactacgagaaacacaaagtctacgcctgcgaagtcacccatcagggcctgagctcgcccgtcacaaagagcttcaacaggggagagtgttaggcggccgctaatcagccataccacatttgtagaggttttacttgctttaaaaaacctcccacacctccccctgaacctgaaacataaaatgaatgcaattgttgttgttaacttgtttattgcagcttataatggttacaaataaagcaatagcatcacaaatttcacaaataaagcatttttttcactgcattctagttgtggtttgtccaaactcatcaatgtatcttatcatgtc

SEQ ID NO: 26 - DNA, 6335 bp, Artificial
  Synthetic plasmid
tcgagctctagattgggaacccgggtctctcgaattcgagatctccaccatgcacagacctagacgtcgtggaactcgtccacctccactggcactgctcgctgctctcctcctggctgcacgtggtgctgatgcagacatccagatgacccagtctccagcctccctgtctgcatctgttggagacagagtcaccatcacttgtcgggcgagtcaggacattagcgattatttagcctggtatcagcagaaaccagggaaaattcctaggctcctgatctatactacatccactttgcaatcaggggtcccatctcggttccgtggcagtgggtctgggacagatttcactctcaccatcagcagcctgcagcctgaagatgttgcaacttattactgtcagaagtatgacagtgccccgctcactttcggcggagggaccaaggtggagatcaaacgaactgtggctgcaccatctgtcttcatcttcccgccatctgatgagcagttgaaatctggaactgcctctgttgtgtgcctgctgaataacttctatcccagagaggccaaagtacagtggaaggtggataacgccctccaatcgggtaactcccaggagagtgtcacagagcaggacagcaaggacagcacctacagcctcagcagcaccctgacgctgagcaaagcagactacgagaaacacaaagtctacgcctgcgaagtcacccatcagggcctgagctcgcccgtcacaaagagcttcaacaggggagagtgttaggcggccgctaatcagccataccacatttgtagaggttttacttgctttaaaaaacctcccacacctccccctgaacctgaaacataaaatgaatgcaattgttgttgttaacttgtttattgcagcttataatggttacaaataaagcaatagcatcacaaatttcacaaataaagcatttttttcactgcattctagttgtggtttgtccaaactcatcaatgtatcttatcatgtctaccggtagggcccctctcttcatgtgagcaaaaggccagcaaaaggccaggaaccgtaaaaaggccgcgttgctggcgtttttccataggctccgcccccctgacgagcatcacaaaaatcgacgctcaagtcagaggtggcgaaacccgacaggactataaagataccaggcgtttccccctggaagctccctcgtgcgctctcctgttccgaccctgccgcttaccggatacctgtccgcctttctcccttcgggaagcgtggcgctttctcaatgctcacgctgtaggtatctcagttcggtgtaggtcgttcgctccaagctgggctgtgtgcacgaaccccccgttcagcccgaccgctgcgccttatccggtaactatcgtcttgagtccaacccggtaagacacgacttatcgccactggcagcagccactggtaacaggattagcagagcgaggtatgtaggcggtgctacagagttcttgaagtggtggcctaactacggctacactagaaggacagtatttggtatctgcgctctgctgaagccagttaccttcggaaaaagagttggtagctcttgatccggcaaacaaaccaccgctggtagcggtggtttttttgtttgcaagcagcagattacgcgcagaaaaaaaggatctcaagaagatcctttgatcttttctacggggtctgacgctcagtggaacgaaaactcacgttaagggattttggtcatgggcgcgggcatgagattatcaaaaaggatcttcacctagatccttttaaattaaaaatgaagttttaaatcaatctaaagtatatatgagtaaacttggtctgacagttaccaatgcttaatcagtgaggcacctatctcagcgatctgtctatttcgttcatccatagttgcctgactccccgtcgtgtagataactacgatacgggagggcttaccatctggccccagtgctgcaatgataccgcgagacccacgctcaccggctccagatttatcagcaataaaccagccagccggaagggccgagcgcagaagtggtcctgcaactttatccgcctccatccagtctattaattgttgccgggaagctagagtaagtagttcgccagttaatagtttgcgcaacgttgttgccattgctacaggcatcgtggtgtcacgctcgtcgtttggtatggcttcattcagctccggttcccaacgatcaaggcgagttacatgatcccccatgttgtgcaaaaaagcggttagctccttcggtcctccgatcgttgtcagaagtaagttggccgcagtgttatcactcatggttatggcagcactgcataattctcttactgtcatgccatccgtaagatgcttttctgtgactggtgagtactcaaccaagtcattctgagaatagtgtatgcggcgaccgagttgctcttgcccggcgtcaatacgggataataccgcgccacatagcagaactttaaaagtgctcatcattggaaaacgttcttcggggcgaaaactctcaaggatcttaccgctgttgagatccagttcgatgtaacccactcgtgcacccaactgatcttcagcatcttttactttcaccagcgtttctgggtgagcaaaaacaggaaggcaaaatgccgcaaaaaagggaataagggcgacacggaaatgttgaatactcatactcttcctttttcaatattattgaagcatttatcagggttattgtctcatgagcggatacatatttgaatgtatttagaaaaataaacaaataggggttccgcgcacatttccccgaaaagtgccacctgacgtcaggtacacttaggcgcgccattagagttcctgcaggctacatggtaccaagcctaggcctccaaaaaagcctcctcactacttctggaatagctcagaggcagaggcggcctcggcctctgcataaataaaaaaaattagtcagccatggggcggagaatgggcggaactgggcggagttaggggcgggatgggcggagttaggggcgggactatggttgctgactaattgagatgcatgctttgcatacttctgcctgctggggagcctggggactttccacacctggttgctgactaattgagatgcatgctttgcatacttctgcctgctggggagcctggggactttccacaccggatccaccatggatagatccggaaagcctgaactcaccgcgacgtctgtcgagaagtttctgatcgaaaagttcgacagcgtctccgacctgatgcagctctcggagggcgaagaatctcgtgctttcagcttcgatgtaggagggcgtggatatgtcctgcgggtaaatagctgcgccgatggtttctacaaagatcgttatgtttatcggcactttgcatcggccgcgctcccgattccggaagtgcttgacattggggagttcagcgagagcctgacctattgcatctcccgccgtgcacagggtgtcacgttgcaagacctgcctgaaaccgaactgcccgctgttctgcagccggtcgcggaggccatggatgcgatcgctgcggccgatcttagccagacgagcgggttcggcccattcggaccgcaaggaatcggtcaatacactacatggcgtgatttcatatgcgcgattgctgatccccatgtgtatcactggcaaactgtgatggacgacaccgtcagtgcgtccgtcgcgcaggctctcgatgagctgatgctttgggccgaggactgccccgaagtccggcacctcgtgcacgcggatttcggctccaacaatgtcctgacggacaatggccgcataacagcggtcattgactggagcgaggcgatgttcggggattcccaatacgaggtcgccaacatcttcttctggaggccgtggttggcttgtatggagcagcagacgcgctacttcgagcggaggcatccggagcttgcaggatcgccgcggctccgggcgtatatgctccgcattggtcttgaccaactctatcagagcttggttgacggcaatttcgatgatgcagcttgggcgcagggtcgatgcgacgcaatcgtccgatccggagccgggactgtcgggcgtacacaaatcgcccgcagaagcgcggccgtctggaccgatggctgtgtagaagtactcgccgatagtggaaaccgacgccccagcactcgtccgagggcaaaggaatagacgcgtgctgtaagtctgcagaaattgatgatctattaaacaataaagatgtccactaaaatggaagtttttcctgtcatactttgttaagaagggtgagaacagagtacctacattttgaatggaaggattggagctacgggggtgggggtggggtgggattagataaatgcctgctctttactgaaggctctttactattgctttatgataatgtttcatagttggatatcataatttaaacaagcaaaaccaaattaagggccagctcattcctcccactcatgatctatggatctatagatctctcgtgcagctggggctctagggggtatccccacgcgccctgtagcggcgcattaagcgcggcgggtgtggtggttacgcgcagcgtgaccgctacacttgccagcgccctagcgcccgctcctttcgctttcttcccttcctttctcgccacgttcgccggctttccccgtcaagctctaaatcgggggctccctttagggttccgatttagtgctttacggcacctcgaccccaaaaaacttgattagggtgatggttcacgtagtgggccatcgccctgatagacggtttttcgccctttgacgttggagtccacgttctttaatagtggactcttgttccaaactggaacaacactcaaccctatctcggtctattcttttgatttataagggattttgccgatttcggcctattggttaaaaaatgagctgatttaacaaaaatttaacgcgaattaattctgtggaatgtgtgtcagttagtcgcgatgtgtgactagttagttattaatagtaatcaattacggggtcattagttcatagcccatatatggagttccgcgttacataacttacggtaaatggcccgcctggctgaccgcccaacgacccccgcccattgacgtcaataatgacgtatgttcccatagtaacgccaatagggactttccattgacgtcaatgggtggagtatttacggtaaactgcccacttggcagtacatcaagtgtatcatatgccaagtacgccccctattgacgtcaatgacggtaaatggcccgcctggcattatgcccagtacatgaccttatgggactttcctacttggcagtacatctacgtattagtcatcgctattaccatggtgatgcggttttggcagtacatcaatgggcgtggatagcggtttgactcacggggatttccaagtctccaccccattgacgtcaatgggagtttgttttggcaccaaaatcaacgggactttccaaaatgtcgtaacaactccgccccattgacgcaaatgggcggtaggcgtgtacggtgggaggtctatataagcagagctcatgatagaagcactctactattcgtcgaccgatcctgagaacttcagggtgagtttggggacccttgattgttctttctttttcgctattgtaaaattcatgttatatggagggggcaaagttttcagggtgttgtttagaatgggaagatgtcccttgtatcaccatggaccctcatgataattttgtttctttcactttctactctgttgacaaccattgtctcctcttattttcttttcattttctgtaactttttcgttaaactttagcttgcatttgtaacgaatttttaaattcacttttgtttatttgtcagattgtaagtactttctctaatcacttttttttcaaggcaatcagggtatattatattgtacttcagcacagttttagagaacaattgttataattaaatgataaggtagaatatttctgcatataaattctggctggcgtggaaatattcttattggtagaaacaactacaccctggtcatcatcctgcctttctctttatggttacaatgatatacactgtttgagatgaggataaaatactctgagtccaaaccgggcccctctgctaaccatgttcatgccttcttctctttcctacagctcctgggcaacgtgctggttgttgtgctgtctcatcattttggcaaagaattaagcttatac

SEQ ID NO: 27 - protein, 452 aa, Homo sapiens
EVQLVESGGGLVQPGGSLRLSCAASGFTFSSYDIHWVRQATGKGLEWVSAIGPAGDTYYPGSVKGRFTISRENAKNSLYLQMNSLRAGDTAVYYCARGLITFGGLIAPFDYWGQGTLVTVSSASTKGPSVFPLAPSSKSTSGGTAALGCLVKDYFPEPVTVSWNSGALTSGVHTFPAVLQSSGLYSLSSVVTVPSSSLGTQTYICNVNHKPSNTKVDKKVEPKSCDKTHTCPPCPAPELLGGPSVFLFPPKPKDTLMISRTPEVTCVVVDVSHEDPEVKFNWYVDGVEVHNAKTKPREEQYNSTYRVVSVLTVLHQDWLNGKEYKCKVSNKALPAPIEKTISKAKGQPREPQVYTLPPSRDELTKNQVSLTCLVKGFYPSDIAVEWESNGQPENNYKTTPPVLDSDGSFFLYSKLTVDKSRWQQGNVFSCSVMHEALHNHYTQKSLSLSPGK

SEQ ID NO: 28 - protein, 112 aa, Homo sapiens
ESGGGLVQPGGSLRLSCAASGFTFSSYDIHWVRQATGKGLEWVSAIGPAGDTYYPGSVKGRFTISRENAKNSLYLQMNSLRAGDTAVYYCARGLITFGGLIAPFDYWGQGTL

SEQ ID NO: 29 - protein, 214 aa, Homo sapiens
EIVLTQSPGTLSLSPGERATLSCRASQSVSSTYLAWYQQKPGQAPRLLIYGASSRATGIPDRFSGSGSGTDFTLTISRLEPEDFAVYYCQHYDNSQTFGQGTKVEIKRTVAAPSVFIFPPSDEQLKSGTASVVCLLNNFYPREAKVQWKVDNALQSGNSQESVTEQDSKDSTYSLSSTLTLSKADYEKHKVYACEVTHQGLSSPVTKSFNRGEC

SEQ ID NO: 30 - protein, 107 aa, Homo sapiens
IVLTQSPGTLSLSPGERATLSCRASQSVSSTYLAWYQQKPGQAPRLLIYGASSRATGIPDRFSGSGSGTDFTLTISRLEPEDFAVYYCQHYDNSQTFGQGTKVEIKR

SEQ ID NO: 31 - DNA, 2986 bp, Artificial
  Synthetic construct
tagttattaatagtaatcaattacggggtcattagttcatagcccatatatggagttccgcgttacataacttacggtaaatggcccgcctggctgaccgcccaacgacccccgcccattgacgtcaataatgacgtatgttcccatagtaacgccaatagggactttccattgacgtcaatgggtggagtatttacggtaaactgcccacttggcagtacatcaagtgtatcatatgccaagtacgccccctattgacgtcaatgacggtaaatggcccgcctggcattatgcccagtacatgaccttatgggactttcctacttggcagtacatctacgtattagtcatcgctattaccatggtgatgcggttttggcagtacatcaatgggcgtggatagcggtttgactcacggggatttccaagtctccaccccattgacgtcaatgggagtttgttttggcaccaaaatcaacgggactttccaaaatgtcgtaacaactccgccccattgacgcaaatgggcggtaggcgtgtacggtgggaggtctatataagcagagctcatgatagaagcactctactattcgtcgaccgatcctgagaacttcagggtgagtttggggacccttgattgttctttctttttcgctattgtaaaattcatgttatatggagggggcaaagttttcagggtgttgtttagaatgggaagatgtcccttgtatcaccatggaccctcatgataattttgtttctttcactttctactctgttgacaaccattgtctcctcttattttcttttcattttctgtaactttttcgttaaactttagcttgcatttgtaacgaatttttaaattcacttttgtttatttgtcagattgtaagtactttctctaatcacttttttttcaaggcaatcagggtatattatattgtacttcagcacagttttagagaacaattgttataattaaatgataaggtagaatatttctgcatataaattctggctggcgtggaaatattcttattggtagaaacaactacaccctggtcatcatcctgcctttctctttatggttacaatgatatacactgtttgagatgaggataaaatactctgagtccaaaccgggcccctctgctaaccatgttcatgccttcttctctttcctacagctcctgggcaacgtgctggttgttgtgctgtctcatcattttggcaaagaattaagcttatactcgagctctagattgggaacccgggtctctcgaattcgagatctccaccatgcacagacctagacgtcgtggaactcgtccacctccactggcactgctcgctgctctcctcctggctgcacgtggtgctgatgcagaggtgcagctggtggagtctgggggaggcttggtacagccgggggggtccctgagactctcctgtgcagcctctggattcaccttcagtagctacgacatacactgggtccgtcaagctacaggaaaaggtctggagtgggtctcagctattggtcctgctggtgacacatactatccaggctccgtgaagggccgattcaccatctccagagaaaatgccaagaactccttgtatcttcaaatgaacagcctgagagccggggacacggctgtgtattactgtgcaagaggtttgattacgtttggggggcttatcgccccgtttgactactggggccagggaaccctggtcaccgtctcctcagcctccaccaagggcccatcggtcttccccctggcaccctcctccaagagcacctctgggggcacagcggccctgggctgcctggtcaaggactacttccccgaaccggtgacggtgtcgtggaactcaggcgccctgaccagcggcgtgcacaccttcccggctgtcctacagtcctcaggactctactccctcagcagcgtggtgaccgtgccctccagcagcttgggcacccagacctacatctgcaacgtgaatcacaagcccagcaacaccaaggtggacaagaaagttgagcccaaatcttgtgacaaaactcacacatgcccaccgtgcccagcacctgaactcctggggggaccgtcagtcttcctcttccccccaaaacccaaggacaccctcatgatctcccggacccctgaggtcacatgcgtggtggtggacgtgagccacgaagaccctgaggtcaagttcaactggtacgtggacggcgtggaggtgcataatgccaagacaaagccgcgggaggagcagtacaacagcacgtaccgtgtggtcagcgtcctcaccgtcctgcaccaggactggctgaatggcaaggagtacaagtgcaaggtctccaacaaagccctcccagcccccatcgagaaaaccatctccaaagccaaagggcagccccgagaaccacaggtgtacaccctgcccccatcccgggatgagctgaccaagaaccaggtcagcctgacctgcctggtcaaaggcttctatcccagcgacatcgccgtggagtgggagagcaatgggcagccggagaacaactacaagaccacgcctcccgtgctggactccgacggctccttcttcctctacagcaagctcaccgtggacaagagcaggtggcagcaggggaacgtcttctcatgctccgtgatgcatgaggctctgcacaaccactacacgcagaagtccctctccctgtctccgggtaaatgagcggccgctaatcagccataccacatttgtagaggttttacttgctttaaaaaacctcccacacctccccctgaacctgaaacataaaatgaatgcaattgttgttgttaacttgtttattgcagcttataatggttacaaataaagcaatagcatcacaaatttcacaaataaagcatttttttcactgcattctagttgtggtttgtccaaactcatcaatgtatcttatcatgtc

SEQ ID NO: 32 - DNA, 7028 bp, Artificial
  Synthetic plasmid
tcgcgatgtgtgactagttagttattaatagtaatcaattacggggtcattagttcatagcccatatatggagttccgcgttacataacttacggtaaatggcccgcctggctgaccgcccaacgacccccgcccattgacgtcaataatgacgtatgttcccatagtaacgccaatagggactttccattgacgtcaatgggtggagtatttacggtaaactgcccacttggcagtacatcaagtgtatcatatgccaagtacgccccctattgacgtcaatgacggtaaatggcccgcctggcattatgcccagtacatgaccttatgggactttcctacttggcagtacatctacgtattagtcatcgctattaccatggtgatgcggttttggcagtacatcaatgggcgtggatagcggtttgactcacggggatttccaagtctccaccccattgacgtcaatgggagtttgttttggcaccaaaatcaacgggactttccaaaatgtcgtaacaactccgccccattgacgcaaatgggcggtaggcgtgtacggtgggaggtctatataagcagagctcatgatagaagcactctactattcgtcgaccgatcctgagaacttcagggtgagtttggggacccttgattgttctttctttttcgctattgtaaaattcatgttatatggagggggcaaagttttcagggtgttgtttagaatgggaagatgtcccttgtatcaccatggaccctcatgataattttgtttctttcactttctactctgttgacaaccattgtctcctcttattttcttttcattttctgtaactttttcgttaaactttagcttgcatttgtaacgaatttttaaattcacttttgtttatttgtcagattgtaagtactttctctaatcacttttttttcaaggcaatcagggtatattatattgtacttcagcacagttttagagaacaattgttataattaaatgataaggtagaatatttctgcatataaattctggctggcgtggaaatattcttattggtagaaacaactacaccctggtcatcatcctgcctttctctttatggttacaatgatatacactgtttgagatgaggataaaatactctgagtccaaaccgggcccctctgctaaccatgttcatgccttcttctctttcctacagctcctgggcaacgtgctggttgttgtgctgtctcatcattttggcaaagaattaagcttatactcgagctctagattgggaacccgggtctctcgaattcgagatctccaccatgcacagacctagacgtcgtggaactcgtccacctccactggcactgctcgctgctctcctcctggctgcacgtggtgctgatgcagaggtgcagctggtggagtctgggggaggcttggtacagccgggggggtccctgagactctcctgtgcagcctctggattcaccttcagtagctacgacatacactgggtccgtcaagctacaggaaaaggtctggagtgggtctcagctattggtcctgctggtgacacatactatccaggctccgtgaagggccgattcaccatctccagagaaaatgccaagaactccttgtatcttcaaatgaacagcctgagagccggggacacggctgtgtattactgtgcaagaggtttgattacgtttggggggcttatcgccccgtttgactactggggccagggaaccctggtcaccgtctcctcagcctccaccaagggcccatcggtcttccccctggcaccctcctccaagagcacctctgggggcacagcggccctgggctgcctggtcaaggactacttccccgaaccggtgacggtgtcgtggaactcaggcgccctgaccagcggcgtgcacaccttcccggctgtcctacagtcctcaggactctactccctcagcagcgtggtgaccgtgccctccagcagcttgggcacccagacctacatctgcaacgtgaatcacaagcccagcaacaccaaggtggacaagaaagttgagcccaaatcttgtgacaaaactcacacatgcccaccgtgcccagcacctgaactcctggggggaccgtcagtcttcctcttccccccaaaacccaaggacaccctcatgatctcccggacccctgaggtcacatgcgtggtggtggacgtgagccacgaagaccctgaggtcaagttcaactggtacgtggacggcgtggaggtgcataatgccaagacaaagccgcgggaggagcagtacaacagcacgtaccgtgtggtcagcgtcctcaccgtcctgcaccaggactggctgaatggcaaggagtacaagtgcaaggtctccaacaaagccctcccagcccccatcgagaaaaccatctccaaagccaaagggcagccccgagaaccacaggtgtacaccctgcccccatcccgggatgagctgaccaagaaccaggtcagcctgacctgcctggtcaaaggcttctatcccagcgacatcgccgtggagtgggagagcaatgggcagccggagaacaactacaagaccacgcctcccgtgctggactccgacggctccttcttcctctacagcaagctcaccgtggacaagagcaggtggcagcaggggaacgtcttctcatgctccgtgatgcatgaggctctgcacaaccactacacgcagaagtccctctccctgtctccgggtaaatgagcggccgctaatcagccataccacatttgtagaggttttacttgctttaaaaaacctcccacacctccccctgaacctgaaacataaaatgaatgcaattgttgttgttaacttgtttattgcagcttataatggttacaaataaagcaatagcatcacaaatttcacaaataaagcatttttttcactgcattctagttgtggtttgtccaaactcatcaatgtatcttatcatgtctaccggtcctgcagggcccctctcttcatgtgagcaaaaggccagcaaaaggccaggaaccgtaaaaaggccgcgttgctggcgtttttccataggctccgcccccctgacgagcatcacaaaaatcgacgctcaagtcagaggtggcgaaacccgacaggactataaagataccaggcgtttccccctggaagctccctcgtgcgctctcctgttccgaccctgccgcttaccggatacctgtccgcctttctcccttcgggaagcgtggcgctttctcaatgctcacgctgtaggtatctcagttcggtgtaggtcgttcgctccaagctgggctgtgtgcacgaaccccccgttcagcccgaccgctgcgccttatccggtaactatcgtcttgagtccaacccggtaagacacgacttatcgccactggcagcagccactggtaacaggattagcagagcgaggtatgtaggcggtgctacagagttcttgaagtggtggcctaactacggctacactagaaggacagtatttggtatctgcgctctgctgaagccagttaccttcggaaaaagagttggtagctcttgatccggcaaacaaaccaccgctggtagcggtggtttttttgtttgcaagcagcagattacgcgcagaaaaaaaggatctcaagaagatcctttgatcttttctacggggtctgacgctcagtggaacgaaaactcacgttaagggattttggtcatgggcgcgcctcatactcctgcaggcatgagattatcaaaaaggatcttcacctagatccttttaaattaaaaatgaagttttaaatcaatctaaagtatatatgagtaaacttggtctgacagttaccaatgcttaatcagtgaggcacctatctcagcgatctgtctatttcgttcatccatagttgcctgactccccgtcgtgtagataactacgatacgggagggcttaccatctggccccagtgctgcaatgataccgcgagacccacgctcaccggctccagatttatcagcaataaaccagccagccggaagggccgagcgcagaagtggtcctgcaactttatccgcctccatccagtctattaattgttgccgggaagctagagtaagtagttcgccagttaatagtttgcgcaacgttgttgccattgctacaggcatcgtggtgtcacgctcgtcgtttggtatggcttcattcagctccggttcccaacgatcaaggcgagttacatgatcccccatgttgtgcaaaaaagcggttagctccttcggtcctccgatcgttgtcagaagtaagttggccgcagtgttatcactcatggttatggcagcactgcataattctcttactgtcatgccatccgtaagatgcttttctgtgactggtgagtactcaaccaagtcattctgagaatagtgtatgcggcgaccgagttgctcttgcccggcgtcaatacgggataataccgcgccacatagcagaactttaaaagtgctcatcattggaaaacgttcttcggggcgaaaactctcaaggatcttaccgctgttgagatccagttcgatgtaacccactcgtgcacccaactgatcttcagcatcttttactttcaccagcgtttctgggtgagcaaaaacaggaaggcaaaatgccgcaaaaaagggaataagggcgacacggaaatgttgaatactcatactcttcctttttcaatattattgaagcatttatcagggttattgtctcatgagcggatacatatttgaatgtatttagaaaaataaacaaataggggttccgcgcacatttccccgaaaagtgccacctgacgtcaggtaccaagcctaggcctccaaaaaagcctcctcactacttctggaatagctcagaggcagaggcggcctcggcctctgcataaataaaaaaaattagtcagccatggggcggagaatgggcggaactgggcggagttaggggcgggatgggcggagttaggggcgggactatggttgctgactaattgagatgcatgctttgcatacttctgcctgctggggagcctggggactttccacacctggttgctgactaattgagatgcatgctttgcatacttctgcctgctggggagcctggggactttccacaccggatccaccatggatagatccggaaagcctgaactcaccgcgacgtctgtcgagaagtttctgatcgaaaagttcgacagcgtctccgacctgatgcagctctcggagggcgaagaatctcgtgctttcagcttcgatgtaggagggcgtggatatgtcctgcgggtaaatagctgcgccgatggtttctacaaagatcgttatgtttatcggcactttgcatcggccgcgctcccgattccggaagtgcttgacattggggagttcagcgagagcctgacctattgcatctcccgccgtgcacagggtgtcacgttgcaagacctgcctgaaaccgaactgcccgctgttctgcagccggtcgcggaggccatggatgcgatcgctgcggccgatcttagccagacgagcgggttcggcccattcggaccgcaaggaatcggtcaatacactacatggcgtgatttcatatgcgcgattgctgatccccatgtgtatcactggcaaactgtgatggacgacaccgtcagtgcgtccgtcgcgcaggctctcgatgagctgatgctttgggccgaggactgccccgaagtccggcacctcgtgcacgcggatttcggctccaacaatgtcctgacggacaatggccgcataacagcggtcattgactggagcgaggcgatgttcggggattcccaatacgaggtcgccaacatcttcttctggaggccgtggttggcttgtatggagcagcagacgcgctacttcgagcggaggcatccggagcttgcaggatcgccgcggctccgggcgtatatgctccgcattggtcttgaccaactctatcagagcttggttgacggcaatttcgatgatgcagcttgggcgcagggtcgatgcgacgcaatcgtccgatccggagccgggactgtcgggcgtacacaaatcgcccgcagaagcgcggccgtctggaccgatggctgtgtagaagtactcgccgatagtggaaaccgacgccccagcactcgtccgagggcaaaggaatagacgcgtgctgtaagtctgcagaaattgatgatctattaaacaataaagatgtccactaaaatggaagtttttcctgtcatactttgttaagaagggtgagaacagagtacctacattttgaatggaaggattggagctacgggggtgggggtggggtgggattagataaatgcctgctctttactgaaggctctttactattgctttatgataatgtttcatagttggatatcataatttaaacaagcaaaaccaaattaagggccagctcattcctcccactcatgatctatggatctatagatctctcgtgcagctggggctctagggggtatccccacgcgccctgtagcggcgcattaagcgcggcgggtgtggtggttacgcgcagcgtgaccgctacacttgccagcgccctagcgcccgctcctttcgctttcttcccttcctttctcgccacgttcgccggctttccccgtcaagctctaaatcgggggctccctttagggttccgatttagtgctttacggcacctcgaccccaaaaaacttgattagggtgatggttcacgtagtgggccatcgccctgatagacggtttttcgccctttgacgttggagtccacgttctttaatagtggactcttgttccaaactggaacaacactcaaccctatctcggtctattcttttgatttataagggattttgccgatttcggcctattggttaaaaaatgagctgatttaacaaaaatttaacgcgaattaattctgtggaatgtgtgtcagttag

SEQ ID NO: 33 - DNA, 2272 bp, Artificial
  Synthetic construct
tagttattaatagtaatcaattacggggtcattagttcatagcccatatatggagttccgcgttacataacttacggtaaatggcccgcctggctgaccgcccaacgacccccgcccattgacgtcaataatgacgtatgttcccatagtaacgccaatagggactttccattgacgtcaatgggtggagtatttacggtaaactgcccacttggcagtacatcaagtgtatcatatgccaagtacgccccctattgacgtcaatgacggtaaatggcccgcctggcattatgcccagtacatgaccttatgggactttcctacttggcagtacatctacgtattagtcatcgctattaccatggtgatgcggttttggcagtacatcaatgggcgtggatagcggtttgactcacggggatttccaagtctccaccccattgacgtcaatgggagtttgttttggcaccaaaatcaacgggactttccaaaatgtcgtaacaactccgccccattgacgcaaatgggcggtaggcgtgtacggtgggaggtctatataagcagagctcatgatagaagcactctactattcgtcgaccgatcctgagaacttcagggtgagtttggggacccttgattgttctttctttttcgctattgtaaaattcatgttatatggagggggcaaagttttcagggtgttgtttagaatgggaagatgtcccttgtatcaccatggaccctcatgataattttgtttctttcactttctactctgttgacaaccattgtctcctcttattttcttttcattttctgtaactttttcgttaaactttagcttgcatttgtaacgaatttttaaattcacttttgtttatttgtcagattgtaagtactttctctaatcacttttttttcaaggcaatcagggtatattatattgtacttcagcacagttttagagaacaattgttataattaaatgataaggtagaatatttctgcatataaattctggctggcgtggaaatattcttattggtagaaacaactacaccctggtcatcatcctgcctttctctttatggttacaatgatatacactgtttgagatgaggataaaatactctgagtccaaaccgggcccctctgctaaccatgttcatgccttcttctctttcctacagctcctgggcaacgtgctggttgttgtgctgtctcatcattttggcaaagaattaagcttatactcgagctctagattgggaacccgggtctctcgaattcgagatctccaccatgcacagacctagacgtcgtggaactcgtccacctccactggcactgctcgctgctctcctcctggctgcacgtggtgctgatgcagaaattgtgttgacgcagtctccaggcaccctgtctttgtctccaggggaaagagccaccctctcctgcagggccagtcagagtgttagcagcacctacttagcctggtaccagcagaaacctggccaggctcccaggctcctcatctatggtgcatccagcagggccactggcatcccagacaggttcagtggcagtgggtctgggacagacttcactctcaccatcagcagactggagcctgaagattttgcagtgtattactgtcagcattatgataactcacaaacgttcggccaagggaccaaggtggagatcaaacgaactgtggctgcaccatctgtcttcatcttcccgccatctgatgagcagttgaaatctggaactgcctctgttgtgtgcctgctgaataacttctatcccagagaggccaaagtacagtggaaggtggataacgccctccaatcgggtaactcccaggagagtgtcacagagcaggacagcaaggacagcacctacagcctcagcagcaccctgacgctgagcaaagcagactacgagaaacacaaagtctacgcctgcgaagtcacccatcagggcctgagctcgcccgtcacaaagagcttcaacaggggagagtgttaggcggccgctaatcagccataccacatttgtagaggttttacttgctttaaaaaacctcccacacctccccctgaacctgaaacataaaatgaatgcaattgttgttgttaacttgtttattgcagcttataatggttacaaataaagcaatagcatcacaaatttcacaaataaagcatttttttcactgcattctagttgtggtttgtccaaactcatcaatgtatcttatcatgtc

SEQ ID NO: 34 - DNA, 6335 bp, Artificial
  Synthetic plasmid
tcgagctctagattgggaacccgggtctctcgaattcgagatctccaccatgcacagacctagacgtcgtggaactcgtccacctccactggcactgctcgctgctctcctcctggctgcacgtggtgctgatgcagaaattgtgttgacgcagtctccaggcaccctgtctttgtctccaggggaaagagccaccctctcctgcagggccagtcagagtgttagcagcacctacttagcctggtaccagcagaaacctggccaggctcccaggctcctcatctatggtgcatccagcagggccactggcatcccagacaggttcagtggcagtgggtctgggacagacttcactctcaccatcagcagactggagcctgaagattttgcagtgtattactgtcagcattatgataactcacaaacgttcggccaagggaccaaggtggagatcaaacgaactgtggctgcaccatctgtcttcatcttcccgccatctgatgagcagttgaaatctggaactgcctctgttgtgtgcctgctgaataacttctatcccagagaggccaaagtacagtggaaggtggataacgccctccaatcgggtaactcccaggagagtgtcacagagcaggacagcaaggacagcacctacagcctcagcagcaccctgacgctgagcaaagcagactacgagaaacacaaagtctacgcctgcgaagtcacccatcagggcctgagctcgcccgtcacaaagagcttcaacaggggagagtgttaggcggccgctaatcagccataccacatttgtagaggttttacttgctttaaaaaacctcccacacctccccctgaacctgaaacataaaatgaatgcaattgttgttgttaacttgtttattgcagcttataatggttacaaataaagcaatagcatcacaaatttcacaaataaagcatttttttcactgcattctagttgtggtttgtccaaactcatcaatgtatcttatcatgtctaccggtagggcccctctcttcatgtgagcaaaaggccagcaaaaggccaggaaccgtaaaaaggccgcgttgctggcgtttttccataggctccgcccccctgacgagcatcacaaaaatcgacgctcaagtcagaggtggcgaaacccgacaggactataaagataccaggcgtttccccctggaagctccctcgtgcgctctcctgttccgaccctgccgcttaccggatacctgtccgcctttctcccttcgggaagcgtggcgctttctcaatgctcacgctgtaggtatctcagttcggtgtaggtcgttcgctccaagctgggctgtgtgcacgaaccccccgttcagcccgaccgctgcgccttatccggtaactatcgtcttgagtccaacccggtaagacacgacttatcgccactggcagcagccactggtaacaggattagcagagcgaggtatgtaggcggtgctacagagttcttgaagtggtggcctaactacggctacactagaaggacagtatttggtatctgcgctctgctgaagccagttaccttcggaaaaagagttggtagctcttgatccggcaaacaaaccaccgctggtagcggtggtttttttgtttgcaagcagcagattacgcgcagaaaaaaaggatctcaagaagatcctttgatcttttctacggggtctgacgctcagtggaacgaaaactcacgttaagggattttggtcatgggcgcgggcatgagattatcaaaaaggatcttcacctagatccttttaaattaaaaatgaagttttaaatcaatctaaagtatatatgagtaaacttggtctgacagttaccaatgcttaatcagtgaggcacctatctcagcgatctgtctatttcgttcatccatagttgcctgactccccgtcgtgtagataactacgatacgggagggcttaccatctggccccagtgctgcaatgataccgcgagacccacgctcaccggctccagatttatcagcaataaaccagccagccggaagggccgagcgcagaagtggtcctgcaactttatccgcctccatccagtctattaattgttgccgggaagctagagtaagtagttcgccagttaatagtttgcgcaacgttgttgccattgctacaggcatcgtggtgtcacgctcgtcgtttggtatggcttcattcagctccggttcccaacgatcaaggcgagttacatgatcccccatgttgtgcaaaaaagcggttagctccttcggtcctccgatcgttgtcagaagtaagttggccgcagtgttatcactcatggttatggcagcactgcataattctcttactgtcatgccatccgtaagatgcttttctgtgactggtgagtactcaaccaagtcattctgagaatagtgtatgcggcgaccgagttgctcttgcccggcgtcaatacgggataataccgcgccacatagcagaactttaaaagtgctcatcattggaaaacgttcttcggggcgaaaactctcaaggatcttaccgctgttgagatccagttcgatgtaacccactcgtgcacccaactgatcttcagcatcttttactttcaccagcgtttctgggtgagcaaaaacaggaaggcaaaatgccgcaaaaaagggaataagggcgacacggaaatgttgaatactcatactcttcctttttcaatattattgaagcatttatcagggttattgtctcatgagcggatacatatttgaatgtatttagaaaaataaacaaataggggttccgcgcacatttccccgaaaagtgccacctgacgtcaggtacacttaggcgcgccattagagttcctgcaggctacatggtaccaagcctaggcctccaaaaaagcctcctcactacttctggaatagctcagaggcagaggcggcctcggcctctgcataaataaaaaaaattagtcagccatggggcggagaatgggcggaactgggcggagttaggggcgggatgggcggagttaggggcgggactatggttgctgactaattgagatgcatgctttgcatacttctgcctgctggggagcctggggactttccacacctggttgctgactaattgagatgcatgctttgcatacttctgcctgctggggagcctggggactttccacaccggatccaccatggatagatccggaaagcctgaactcaccgcgacgtctgtcgagaagtttctgatcgaaaagttcgacagcgtctccgacctgatgcagctctcggagggcgaagaatctcgtgctttcagcttcgatgtaggagggcgtggatatgtcctgcgggtaaatagctgcgccgatggtttctacaaagatcgttatgtttatcggcactttgcatcggccgcgctcccgattccggaagtgcttgacattggggagttcagcgagagcctgacctattgcatctcccgccgtgcacagggtgtcacgttgcaagacctgcctgaaaccgaactgcccgctgttctgcagccggtcgcggaggccatggatgcgatcgctgcggccgatcttagccagacgagcgggttcggcccattcggaccgcaaggaatcggtcaatacactacatggcgtgatttcatatgcgcgattgctgatccccatgtgtatcactggcaaactgtgatggacgacaccgtcagtgcgtccgtcgcgcaggctctcgatgagctgatgctttgggccgaggactgccccgaagtccggcacctcgtgcacgcggatttcggctccaacaatgtcctgacggacaatggccgcataacagcggtcattgactggagcgaggcgatgttcggggattcccaatacgaggtcgccaacatcttcttctggaggccgtggttggcttgtatggagcagcagacgcgctacttcgagcggaggcatccggagcttgcaggatcgccgcggctccgggcgtatatgctccgcattggtcttgaccaactctatcagagcttggttgacggcaatttcgatgatgcagcttgggcgcagggtcgatgcgacgcaatcgtccgatccggagccgggactgtcgggcgtacacaaatcgcccgcagaagcgcggccgtctggaccgatggctgtgtagaagtactcgccgatagtggaaaccgacgccccagcactcgtccgagggcaaaggaatagacgcgtgctgtaagtctgcagaaattgatgatctattaaacaataaagatgtccactaaaatggaagtttttcctgtcatactttgttaagaagggtgagaacagagtacctacattttgaatggaaggattggagctacgggggtgggggtggggtgggattagataaatgcctgctctttactgaaggctctttactattgctttatgataatgtttcatagttggatatcataatttaaacaagcaaaaccaaattaagggccagctcattcctcccactcatgatctatggatctatagatctctcgtgcagctggggctctagggggtatccccacgcgccctgtagcggcgcattaagcgcggcgggtgtggtggttacgcgcagcgtgaccgctacacttgccagcgccctagcgcccgctcctttcgctttcttcccttcctttctcgccacgttcgccggctttccccgtcaagctctaaatcgggggctccctttagggttccgatttagtgctttacggcacctcgaccccaaaaaacttgattagggtgatggttcacgtagtgggccatcgccctgatagacggtttttcgccctttgacgttggagtccacgttctttaatagtggactcttgttccaaactggaacaacactcaaccctatctcggtctattcttttgatttataagggattttgccgatttcggcctattggttaaaaaatgagctgatttaacaaaaatttaacgcgaattaattctgtggaatgtgtgtcagttagtcgcgatgtgtgactagttagttattaatagtaatcaattacggggtcattagttcatagcccatatatggagttccgcgttacataacttacggtaaatggcccgcctggctgaccgcccaacgacccccgcccattgacgtcaataatgacgtatgttcccatagtaacgccaatagggactttccattgacgtcaatgggtggagtatttacggtaaactgcccacttggcagtacatcaagtgtatcatatgccaagtacgccccctattgacgtcaatgacggtaaatggcccgcctggcattatgcccagtacatgaccttatgggactttcctacttggcagtacatctacgtattagtcatcgctattaccatggtgatgcggttttggcagtacatcaatgggcgtggatagcggtttgactcacggggatttccaagtctccaccccattgacgtcaatgggagtttgttttggcaccaaaatcaacgggactttccaaaatgtcgtaacaactccgccccattgacgcaaatgggcggtaggcgtgtacggtgggaggtctatataagcagagctcatgatagaagcactctactattcgtcgaccgatcctgagaacttcagggtgagtttggggacccttgattgttctttctttttcgctattgtaaaattcatgttatatggagggggcaaagttttcagggtgttgtttagaatgggaagatgtcccttgtatcaccatggaccctcatgataattttgtttctttcactttctactctgttgacaaccattgtctcctcttattttcttttcattttctgtaactttttcgttaaactttagcttgcatttgtaacgaatttttaaattcacttttgtttatttgtcagattgtaagtactttctctaatcacttttttttcaaggcaatcagggtatattatattgtacttcagcacagttttagagaacaattgttataattaaatgataaggtagaatatttctgcatataaattctggctggcgtggaaatattcttattggtagaaacaactacaccctggtcatcatcctgcctttctctttatggttacaatgatatacactgtttgagatgaggataaaatactctgagtccaaaccgggcccctctgctaaccatgttcatgccttcttctctttcctacagctcctgggcaacgtgctggttgttgtgctgtctcatcattttggcaaagaattaagcttatac

SEQ ID NO: 35 - protein, 449 aa, Homo sapiens
QVQLQQSGAGLLKPSETLSLTCTVYGGSFSIHHWTWIRHPPGKGLEWIGEINHRGSTNYNPSLKSRVTISIDTSKNQFSLKLSAVTAADTAVYYCARGLRFLDWLSSYFDYWGQGTLVTVSSASTKGPSVFPLAPCSRSTSESTAALGCLVKDYFPEPVTVSWNSGALTSGVHTFPAVLQSSGLYSLSSVVTVPSSSLGTKTYTCNVDHKPSNTKVDKRVESKYGPPCPPCPAPEFLGGPSVFLFPPKPKDTLMISRTPEVTCVVVDVSQEDPEVQFNWYVDGVEVHNAKTKPREEQFNSTYRVVSVLTVLHQDWLNGKEYKCKVSNKGLPSSIEKTISKAKGQPREPQVYTLPPSQEEMTKNQVSLTCLVKGFYPSDIAVEWESNGQPENNYKTTPPVLDSDGSFFLYSRLTVDKSRWQEGNVFSCSVMHEALHNHYTQKSLSLSLGK

SEQ ID NO: 36 - protein, 103 aa, Homo sapiens
QSGAGLLKPSETLSLTCTVYGGSFSIHHWTWIRHPPGKGLEWIGEINHRGSTNYNPSLKSRVTISIDTSKNQFSLKLSAVTAADTAVYYCARGLRFLDWLSSY

SEQ ID NO: 37 - protein, 214 aa, Homo sapiens
DIQMTQSPSSLSASVGDRVTITCRASQGISDYLAWYQQKPGKVPNLLIYAASALQSGVPSRFSGSGSGTDFTLTISSLQPEDVATYYCQNYNTAPLTFGGGTKVEIKRTVAAPSVFIFPPSDEQLKSGTASVVCLLNNFYPREAKVQWKVDNALQSGNSQESVTEQDSKDSTYSLSSTLTLSKADYEKHKVYACEVTHQGLSSPVTKSFNRGEC

SEQ ID NO: 38 - protein, 107 aa, Homo sapiens
IQMTQSPSSLSASVGDRVTITCRASQGISDYLAWYQQKPGKVPNLLIYAASALQSGVPSRFSGSGSGTDFTLTISSLQPEDVATYYCQNYNTAPLTFGGGTKVEIKR

SEQ ID NO: 39 - DNA, 2977 bp, Artificial
  Synthetic construct
tagttattaatagtaatcaattacggggtcattagttcatagcccatatatggagttccgcgttacataacttacggtaaatggcccgcctggctgaccgcccaacgacccccgcccattgacgtcaataatgacgtatgttcccatagtaacgccaatagggactttccattgacgtcaatgggtggagtatttacggtaaactgcccacttggcagtacatcaagtgtatcatatgccaagtacgccccctattgacgtcaatgacggtaaatggcccgcctggcattatgcccagtacatgaccttatgggactttcctacttggcagtacatctacgtattagtcatcgctattaccatggtgatgcggttttggcagtacatcaatgggcgtggatagcggtttgactcacggggatttccaagtctccaccccattgacgtcaatgggagtttgttttggcaccaaaatcaacgggactttccaaaatgtcgtaacaactccgccccattgacgcaaatgggcggtaggcgtgtacggtgggaggtctatataagcagagctcatgatagaagcactctactattcgtcgaccgatcctgagaacttcagggtgagtttggggacccttgattgttctttctttttcgctattgtaaaattcatgttatatggagggggcaaagttttcagggtgttgtttagaatgggaagatgtcccttgtatcaccatggaccctcatgataattttgtttctttcactttctactctgttgacaaccattgtctcctcttattttcttttcattttctgtaactttttcgttaaactttagcttgcatttgtaacgaatttttaaattcacttttgtttatttgtcagattgtaagtactttctctaatcacttttttttcaaggcaatcagggtatattatattgtacttcagcacagttttagagaacaattgttataattaaatgataaggtagaatatttctgcatataaattctggctggcgtggaaatattcttattggtagaaacaactacaccctggtcatcatcctgcctttctctttatggttacaatgatatacactgtttgagatgaggataaaatactctgagtccaaaccgggcccctctgctaaccatgttcatgccttcttctctttcctacagctcctgggcaacgtgctggttgttgtgctgtctcatcattttggcaaagaattaagcttatactcgagctctagattgggaacccgggtctctcgaattcgagatctccaccatgcacagacctagacgtcgtggaactcgtccacctccactggcactgctcgctgctctcctcctggctgcacgtggtgctgatgcacaggtacagctgcagcagtcgggcgcaggactgttgaagccttcggagaccctgtccctcacctgcactgtctatggtggatccttcagtattcatcactggacctggatccgccatcccccagggaaggggctggagtggattggggagatcaatcatcgtggaagcaccaactacaacccgtccctcaagagtcgagtcaccatatcaatagacacgtccaagaaccagttctccctgaagctgagcgctgtgaccgccgcggacacggctgtatattactgtgcgagaggcttacgatttttggactggttatcgtcctactttgactactggggccagggaaccctggtcaccgtctcctcagcctccaccaagggcccatcggtcttccccctggcgccctgctccaggagcacctccgagagcacagccgccctgggctgcctggtcaaggactacttccccgaaccggtgacggtgtcgtggaactcaggcgccctgaccagcggcgtgcacaccttcccggctgtcctacagtcctcaggactctactccctcagcagcgtggtgaccgtgccctccagcagcttgggcacgaagacctacacctgcaacgtagatcacaagcccagcaacaccaaggtggacaagagagttgagtccaaatatggtcccccatgcccaccctgcccagcacctgagttcctggggggaccatcagtcttcctgttccccccaaaacccaaggacactctcatgatctcccggacccctgaggtcacgtgcgtggtggtggacgtgagccaggaagaccccgaggtccagttcaactggtacgtggatggcgtggaggtgcataatgccaagacaaagccgcgggaggagcagttcaacagcacgtaccgtgtggtcagcgtcctcaccgtcctgcaccaggactggctgaacggcaaggagtacaagtgcaaggtctccaacaaaggcctcccgtcctccatcgagaaaaccatctccaaagccaaagggcagccccgagagccacaggtgtacaccctgcccccatcccaggaggagatgaccaagaaccaggtcagcctgacctgcctggtcaaaggcttctaccccagcgacatcgccgtggagtgggagagcaatgggcagccggagaacaactacaagaccacgcctcccgtgctggactccgacggctccttcttcctctacagcaggctcaccgtggacaagagcaggtggcaggaggggaatgtcttctcatgctccgtgatgcatgaggctctgcacaaccactacacacagaagtccctctccctgtctctgggtaaatgagcggccgctaatcagccataccacatttgtagaggttttacttgctttaaaaaacctcccacacctccccctgaacctgaaacataaaatgaatgcaattgttgttgttaacttgtttattgcagcttataatggttacaaataaagcaatagcatcacaaatttcacaaataaagcatttttttcactgcattctagttgtggtttgtccaaactcatcaatgtatcttatcatgtc

SEQ ID NO: 40 - DNA, 7019 bp, Artificial
  Synthetic plasmid
tcgcgatgtgtgactagttagttattaatagtaatcaattacggggtcattagttcatagcccatatatggagttccgcgttacataacttacggtaaatggcccgcctggctgaccgcccaacgacccccgcccattgacgtcaataatgacgtatgttcccatagtaacgccaatagggactttccattgacgtcaatgggtggagtatttacggtaaactgcccacttggcagtacatcaagtgtatcatatgccaagtacgccccctattgacgtcaatgacggtaaatggcccgcctggcattatgcccagtacatgaccttatgggactttcctacttggcagtacatctacgtattagtcatcgctattaccatggtgatgcggttttggcagtacatcaatgggcgtggatagcggtttgactcacggggatttccaagtctccaccccattgacgtcaatgggagtttgttttggcaccaaaatcaacgggactttccaaaatgtcgtaacaactccgccccattgacgcaaatgggcggtaggcgtgtacggtgggaggtctatataagcagagctcatgatagaagcactctactattcgtcgaccgatcctgagaacttcagggtgagtttggggacccttgattgttctttctttttcgctattgtaaaattcatgttatatggagggggcaaagttttcagggtgttgtttagaatgggaagatgtcccttgtatcaccatggaccctcatgataattttgtttctttcactttctactctgttgacaaccattgtctcctcttattttcttttcattttctgtaactttttcgttaaactttagcttgcatttgtaacgaatttttaaattcacttttgtttatttgtcagattgtaagtactttctctaatcacttttttttcaaggcaatcagggtatattatattgtacttcagcacagttttagagaacaattgttataattaaatgataaggtagaatatttctgcatataaattctggctggcgtggaaatattcttattggtagaaacaactacaccctggtcatcatcctgcctttctctttatggttacaatgatatacactgtttgagatgaggataaaatactctgagtccaaaccgggcccctctgctaaccatgttcatgccttcttctctttcctacagctcctgggcaacgtgctggttgttgtgctgtctcatcattttggcaaagaattaagcttatactcgagctctagattgggaacccgggtctctcgaattcgagatctccaccatgcacagacctagacgtcgtggaactcgtccacctccactggcactgctcgctgctctcctcctggctgcacgtggtgctgatgcacaggtacagctgcagcagtcgggcgcaggactgttgaagccttcggagaccctgtccctcacctgcactgtctatggtggatccttcagtattcatcactggacctggatccgccatcccccagggaaggggctggagtggattggggagatcaatcatcgtggaagcaccaactacaacccgtccctcaagagtcgagtcaccatatcaatagacacgtccaagaaccagttctccctgaagctgagcgctgtgaccgccgcggacacggctgtatattactgtgcgagaggcttacgatttttggactggttatcgtcctactttgactactggggccagggaaccctggtcaccgtctcctcagcctccaccaagggcccatcggtcttccccctggcgccctgctccaggagcacctccgagagcacagccgccctgggctgcctggtcaaggactacttccccgaaccggtgacggtgtcgtggaactcaggcgccctgaccagcggcgtgcacaccttcccggctgtcctacagtcctcaggactctactccctcagcagcgtggtgaccgtgccctccagcagcttgggcacgaagacctacacctgcaacgtagatcacaagcccagcaacaccaaggtggacaagagagttgagtccaaatatggtcccccatgcccaccctgcccagcacctgagttcctggggggaccatcagtcttcctgttccccccaaaacccaaggacactctcatgatctcccggacccctgaggtcacgtgcgtggtggtggacgtgagccaggaagaccccgaggtccagttcaactggtacgtggatggcgtggaggtgcataatgccaagacaaagccgcgggaggagcagttcaacagcacgtaccgtgtggtcagcgtcctcaccgtcctgcaccaggactggctgaacggcaaggagtacaagtgcaaggtctccaacaaaggcctcccgtcctccatcgagaaaaccatctccaaagccaaagggcagccccgagagccacaggtgtacaccctgcccccatcccaggaggagatgaccaagaaccaggtcagcctgacctgcctggtcaaaggcttctaccccagcgacatcgccgtggagtgggagagcaatgggcagccggagaacaactacaagaccacgcctcccgtgctggactccgacggctccttcttcctctacagcaggctcaccgtggacaagagcaggtggcaggaggggaatgtcttctcatgctccgtgatgcatgaggctctgcacaaccactacacacagaagtccctctccctgtctctgggtaaatgagcggccgctaatcagccataccacatttgtagaggttttacttgctttaaaaaacctcccacacctccccctgaacctgaaacataaaatgaatgcaattgttgttgttaacttgtttattgcagcttataatggttacaaataaagcaatagcatcacaaatttcacaaataaagcatttttttcactgcattctagttgtggtttgtccaaactcatcaatgtatcttatcatgtctaccggtcctgcagggcccctctcttcatgtgagcaaaaggccagcaaaaggccaggaaccgtaaaaaggccgcgttgctggcgtttttccataggctccgcccccctgacgagcatcacaaaaatcgacgctcaagtcagaggtggcgaaacccgacaggactataaagataccaggcgtttccccctggaagctccctcgtgcgctctcctgttccgaccctgccgcttaccggatacctgtccgcctttctcccttcgggaagcgtggcgctttctcaatgctcacgctgtaggtatctcagttcggtgtaggtcgttcgctccaagctgggctgtgtgcacgaaccccccgttcagcccgaccgctgcgccttatccggtaactatcgtcttgagtccaacccggtaagacacgacttatcgccactggcagcagccactggtaacaggattagcagagcgaggtatgtaggcggtgctacagagttcttgaagtggtggcctaactacggctacactagaaggacagtatttggtatctgcgctctgctgaagccagttaccttcggaaaaagagttggtagctcttgatccggcaaacaaaccaccgctggtagcggtggtttttttgtttgcaagcagcagattacgcgcagaaaaaaaggatctcaagaagatcctttgatcttttctacggggtctgacgctcagtggaacgaaaactcacgttaagggattttggtcatgggcgcgcctcatactcctgcaggcatgagattatcaaaaaggatcttcacctagatccttttaaattaaaaatgaagttttaaatcaatctaaagtatatatgagtaaacttggtctgacagttaccaatgcttaatcagtgaggcacctatctcagcgatctgtctatttcgttcatccatagttgcctgactccccgtcgtgtagataactacgatacgggagggcttaccatctggccccagtgctgcaatgataccgcgagacccacgctcaccggctccagatttatcagcaataaaccagccagccggaagggccgagcgcagaagtggtcctgcaactttatccgcctccatccagtctattaattgttgccgggaagctagagtaagtagttcgccagttaatagtttgcgcaacgttgttgccattgctacaggcatcgtggtgtcacgctcgtcgtttggtatggcttcattcagctccggttcccaacgatcaaggcgagttacatgatcccccatgttgtgcaaaaaagcggttagctccttcggtcctccgatcgttgtcagaagtaagttggccgcagtgttatcactcatggttatggcagcactgcataattctcttactgtcatgccatccgtaagatgcttttctgtgactggtgagtactcaaccaagtcattctgagaatagtgtatgcggcgaccgagttgctcttgcccggcgtcaatacgggataataccgcgccacatagcagaactttaaaagtgctcatcattggaaaacgttcttcggggcgaaaactctcaaggatcttaccgctgttgagatccagttcgatgtaacccactcgtgcacccaactgatcttcagcatcttttactttcaccagcgtttctgggtgagcaaaaacaggaaggcaaaatgccgcaaaaaagggaataagggcgacacggaaatgttgaatactcatactcttcctttttcaatattattgaagcatttatcagggttattgtctcatgagcggatacatatttgaatgtatttagaaaaataaacaaataggggttccgcgcacatttccccgaaaagtgccacctgacgtcaggtaccaagcctaggcctccaaaaaagcctcctcactacttctggaatagctcagaggcagaggcggcctcggcctctgcataaataaaaaaaattagtcagccatggggcggagaatgggcggaactgggcggagttaggggcgggatgggcggagttaggggcgggactatggttgctgactaattgagatgcatgctttgcatacttctgcctgctggggagcctggggactttccacacctggttgctgactaattgagatgcatgctttgcatacttctgcctgctggggagcctggggactttccacaccggatccaccatggatagatccggaaagcctgaactcaccgcgacgtctgtcgagaagtttctgatcgaaaagttcgacagcgtctccgacctgatgcagctctcggagggcgaagaatctcgtgctttcagcttcgatgtaggagggcgtggatatgtcctgcgggtaaatagctgcgccgatggtttctacaaagatcgttatgtttatcggcactttgcatcggccgcgctcccgattccggaagtgcttgacattggggagttcagcgagagcctgacctattgcatctcccgccgtgcacagggtgtcacgttgcaagacctgcctgaaaccgaactgcccgctgttctgcagccggtcgcggaggccatggatgcgatcgctgcggccgatcttagccagacgagcgggttcggcccattcggaccgcaaggaatcggtcaatacactacatggcgtgatttcatatgcgcgattgctgatccccatgtgtatcactggcaaactgtgatggacgacaccgtcagtgcgtccgtcgcgcaggctctcgatgagctgatgctttgggccgaggactgccccgaagtccggcacctcgtgcacgcggatttcggctccaacaatgtcctgacggacaatggccgcataacagcggtcattgactggagcgaggcgatgttcggggattcccaatacgaggtcgccaacatcttcttctggaggccgtggttggcttgtatggagcagcagacgcgctacttcgagcggaggcatccggagcttgcaggatcgccgcggctccgggcgtatatgctccgcattggtcttgaccaactctatcagagcttggttgacggcaatttcgatgatgcagcttgggcgcagggtcgatgcgacgcaatcgtccgatccggagccgggactgtcgggcgtacacaaatcgcccgcagaagcgcggccgtctggaccgatggctgtgtagaagtactcgccgatagtggaaaccgacgccccagcactcgtccgagggcaaaggaatagacgcgtgctgtaagtctgcagaaattgatgatctattaaacaataaagatgtccactaaaatggaagtttttcctgtcatactttgttaagaagggtgagaacagagtacctacattttgaatggaaggattggagctacgggggtgggggtggggtgggattagataaatgcctgctctttactgaaggctctttactattgctttatgataatgtttcatagttggatatcataatttaaacaagcaaaaccaaattaagggccagctcattcctcccactcatgatctatggatctatagatctctcgtgcagctggggctctagggggtatccccacgcgccctgtagcggcgcattaagcgcggcgggtgtggtggttacgcgcagcgtgaccgctacacttgccagcgccctagcgcccgctcctttcgctttcttcccttcctttctcgccacgttcgccggctttccccgtcaagctctaaatcgggggctccctttagggttccgatttagtgctttacggcacctcgaccccaaaaaacttgattagggtgatggttcacgtagtgggccatcgccctgatagacggtttttcgccctttgacgttggagtccacgttctttaatagtggactcttgttccaaactggaacaacactcaaccctatctcggtctattcttttgatttataagggattttgccgatttcggcctattggttaaaaaatgagctgatttaacaaaaatttaacgcgaattaattctgtggaatgtgtgtcagttag

SEQ ID NO: 41 - DNA, 2272 bp, Artificial
  Synthetic construct
tagttattaatagtaatcaattacggggtcattagttcatagcccatatatggagttccgcgttacataacttacggtaaatggcccgcctggctgaccgcccaacgacccccgcccattgacgtcaataatgacgtatgttcccatagtaacgccaatagggactttccattgacgtcaatgggtggagtatttacggtaaactgcccacttggcagtacatcaagtgtatcatatgccaagtacgccccctattgacgtcaatgacggtaaatggcccgcctggcattatgcccagtacatgaccttatgggactttcctacttggcagtacatctacgtattagtcatcgctattaccatggtgatgcggttttggcagtacatcaatgggcgtggatagcggtttgactcacggggatttccaagtctccaccccattgacgtcaatgggagtttgttttggcaccaaaatcaacgggactttccaaaatgtcgtaacaactccgccccattgacgcaaatgggcggtaggcgtgtacggtgggaggtctatataagcagagctcatgatagaagcactctactattcgtcgaccgatcctgagaacttcagggtgagtttggggacccttgattgttctttctttttcgctattgtaaaattcatgttatatggagggggcaaagttttcagggtgttgtttagaatgggaagatgtcccttgtatcaccatggaccctcatgataattttgtttctttcactttctactctgttgacaaccattgtctcctcttattttcttttcattttctgtaactttttcgttaaactttagcttgcatttgtaacgaatttttaaattcacttttgtttatttgtcagattgtaagtactttctctaatcacttttttttcaaggcaatcagggtatattatattgtacttcagcacagttttagagaacaattgttataattaaatgataaggtagaatatttctgcatataaattctggctggcgtggaaatattcttattggtagaaacaactacaccctggtcatcatcctgcctttctctttatggttacaatgatatacactgtttgagatgaggataaaatactctgagtccaaaccgggcccctctgctaaccatgttcatgccttcttctctttcctacagctcctgggcaacgtgctggttgttgtgctgtctcatcattttggcaaagaattaagcttatactcgagctctagattgggaacccgggtctctcgaattcgagatctccaccatgcacagacctagacgtcgtggaactcgtccacctccactggcactgctcgctgctctcctcctggctgcacgtggtgctgatgcagacatccagatgacccagtctccatcctccctgtctgcatctgtaggagacagagtcaccatcacttgccgggcgagtcagggcattagcgattatttagcctggtatcagcagaaaccagggaaagttcctaacctcctgatctatgctgcgtccgctttacaatcaggggtcccatctcgtttcagtggcagtggatctgggacagatttcactctcaccatcagcagcctgcagcctgaggatgttgcaacttattactgtcaaaattataacactgccccgctcactttcggcggggggaccaaggtggaaatcaaacgaactgtggctgcaccatctgtcttcatcttcccgccatctgatgagcagttgaaatctggaactgcctctgttgtgtgcctgctgaataacttctatcccagagaggccaaagtacagtggaaggtggataacgccctccaatcgggtaactcccaggagagtgtcacagagcaggacagcaaggacagcacctacagcctcagcagcaccctgacgctgagcaaagcagactacgagaaacacaaagtctacgcctgcgaagtcacccatcagggcctgagctcgcccgtcacaaagagcttcaacaggggagagtgttaggcggccgctaatcagccataccacatttgtagaggttttacttgctttaaaaaacctcccacacctccccctgaacctgaaacataaaatgaatgcaattgttgttgttaacttgtttattgcagcttataatggttacaaataaagcaatagcatcacaaatttcacaaataaagcatttttttcactgcattctagttgtggtttgtccaaactcatcaatgtatcttatcatgtc

SEQ ID NO: 42 - DNA, 6335 bp, Artificial
  Synthetic plasmid
tcgagctctagattgggaacccgggtctctcgaattcgagatctccaccatgcacagacctagacgtcgtggaactcgtccacctccactggcactgctcgctgctctcctcctggctgcacgtggtgctgatgcagacatccagatgacccagtctccatcctccctgtctgcatctgtaggagacagagtcaccatcacttgccgggcgagtcagggcattagcgattatttagcctggtatcagcagaaaccagggaaagttcctaacctcctgatctatgctgcgtccgctttacaatcaggggtcccatctcgtttcagtggcagtggatctgggacagatttcactctcaccatcagcagcctgcagcctgaggatgttgcaacttattactgtcaaaattataacactgccccgctcactttcggcggggggaccaaggtggaaatcaaacgaactgtggctgcaccatctgtcttcatcttcccgccatctgatgagcagttgaaatctggaactgcctctgttgtgtgcctgctgaataacttctatcccagagaggccaaagtacagtggaaggtggataacgccctccaatcgggtaactcccaggagagtgtcacagagcaggacagcaaggacagcacctacagcctcagcagcaccctgacgctgagcaaagcagactacgagaaacacaaagtctacgcctgcgaagtcacccatcagggcctgagctcgcccgtcacaaagagcttcaacaggggagagtgttaggcggccgctaatcagccataccacatttgtagaggttttacttgctttaaaaaacctcccacacctccccctgaacctgaaacataaaatgaatgcaattgttgttgttaacttgtttattgcagcttataatggttacaaataaagcaatagcatcacaaatttcacaaataaagcatttttttcactgcattctagttgtggtttgtccaaactcatcaatgtatcttatcatgtctaccggtagggcccctctcttcatgtgagcaaaaggccagcaaaaggccaggaaccgtaaaaaggccgcgttgctggcgtttttccataggctccgcccccctgacgagcatcacaaaaatcgacgctcaagtcagaggtggcgaaacccgacaggactataaagataccaggcgtttccccctggaagctccctcgtgcgctctcctgttccgaccctgccgcttaccggatacctgtccgcctttctcccttcgggaagcgtggcgctttctcaatgctcacgctgtaggtatctcagttcggtgtaggtcgttcgctccaagctgggctgtgtgcacgaaccccccgttcagcccgaccgctgcgccttatccggtaactatcgtcttgagtccaacccggtaagacacgacttatcgccactggcagcagccactggtaacaggattagcagagcgaggtatgtaggcggtgctacagagttcttgaagtggtggcctaactacggctacactagaaggacagtatttggtatctgcgctctgctgaagccagttaccttcggaaaaagagttggtagctcttgatccggcaaacaaaccaccgctggtagcggtggtttttttgtttgcaagcagcagattacgcgcagaaaaaaaggatctcaagaagatcctttgatcttttctacggggtctgacgctcagtggaacgaaaactcacgttaagggattttggtcatgggcgcgggcatgagattatcaaaaaggatcttcacctagatccttttaaattaaaaatgaagttttaaatcaatctaaagtatatatgagtaaacttggtctgacagttaccaatgcttaatcagtgaggcacctatctcagcgatctgtctatttcgttcatccatagttgcctgactccccgtcgtgtagataactacgatacgggagggcttaccatctggccccagtgctgcaatgataccgcgagacccacgctcaccggctccagatttatcagcaataaaccagccagccggaagggccgagcgcagaagtggtcctgcaactttatccgcctccatccagtctattaattgttgccgggaagctagagtaagtagttcgccagttaatagtttgcgcaacgttgttgccattgctacaggcatcgtggtgtcacgctcgtcgtttggtatggcttcattcagctccggttcccaacgatcaaggcgagttacatgatcccccatgttgtgcaaaaaagcggttagctccttcggtcctccgatcgttgtcagaagtaagttggccgcagtgttatcactcatggttatggcagcactgcataattctcttactgtcatgccatccgtaagatgcttttctgtgactggtgagtactcaaccaagtcattctgagaatagtgtatgcggcgaccgagttgctcttgcccggcgtcaatacgggataataccgcgccacatagcagaactttaaaagtgctcatcattggaaaacgttcttcggggcgaaaactctcaaggatcttaccgctgttgagatccagttcgatgtaacccactcgtgcacccaactgatcttcagcatcttttactttcaccagcgtttctgggtgagcaaaaacaggaaggcaaaatgccgcaaaaaagggaataagggcgacacggaaatgttgaatactcatactcttcctttttcaatattattgaagcatttatcagggttattgtctcatgagcggatacatatttgaatgtatttagaaaaataaacaaataggggttccgcgcacatttccccgaaaagtgccacctgacgtcaggtacacttaggcgcgccattagagttcctgcaggctacatggtaccaagcctaggcctccaaaaaagcctcctcactacttctggaatagctcagaggcagaggcggcctcggcctctgcataaataaaaaaaattagtcagccatggggcggagaatgggcggaactgggcggagttaggggcgggatgggcggagttaggggcgggactatggttgctgactaattgagatgcatgctttgcatacttctgcctgctggggagcctggggactttccacacctggttgctgactaattgagatgcatgctttgcatacttctgcctgctggggagcctggggactttccacaccggatccaccatggatagatccggaaagcctgaactcaccgcgacgtctgtcgagaagtttctgatcgaaaagttcgacagcgtctccgacctgatgcagctctcggagggcgaagaatctcgtgctttcagcttcgatgtaggagggcgtggatatgtcctgcgggtaaatagctgcgccgatggtttctacaaagatcgttatgtttatcggcactttgcatcggccgcgctcccgattccggaagtgcttgacattggggagttcagcgagagcctgacctattgcatctcccgccgtgcacagggtgtcacgttgcaagacctgcctgaaaccgaactgcccgctgttctgcagccggtcgcggaggccatggatgcgatcgctgcggccgatcttagccagacgagcgggttcggcccattcggaccgcaaggaatcggtcaatacactacatggcgtgatttcatatgcgcgattgctgatccccatgtgtatcactggcaaactgtgatggacgacaccgtcagtgcgtccgtcgcgcaggctctcgatgagctgatgctttgggccgaggactgccccgaagtccggcacctcgtgcacgcggatttcggctccaacaatgtcctgacggacaatggccgcataacagcggtcattgactggagcgaggcgatgttcggggattcccaatacgaggtcgccaacatcttcttctggaggccgtggttggcttgtatggagcagcagacgcgctacttcgagcggaggcatccggagcttgcaggatcgccgcggctccgggcgtatatgctccgcattggtcttgaccaactctatcagagcttggttgacggcaatttcgatgatgcagcttgggcgcagggtcgatgcgacgcaatcgtccgatccggagccgggactgtcgggcgtacacaaatcgcccgcagaagcgcggccgtctggaccgatggctgtgtagaagtactcgccgatagtggaaaccgacgccccagcactcgtccgagggcaaaggaatagacgcgtgctgtaagtctgcagaaattgatgatctattaaacaataaagatgtccactaaaatggaagtttttcctgtcatactttgttaagaagggtgagaacagagtacctacattttgaatggaaggattggagctacgggggtgggggtggggtgggattagataaatgcctgctctttactgaaggctctttactattgctttatgataatgtttcatagttggatatcataatttaaacaagcaaaaccaaattaagggccagctcattcctcccactcatgatctatggatctatagatctctcgtgcagctggggctctagggggtatccccacgcgccctgtagcggcgcattaagcgcggcgggtgtggtggttacgcgcagcgtgaccgctacacttgccagcgccctagcgcccgctcctttcgctttcttcccttcctttctcgccacgttcgccggctttccccgtcaagctctaaatcgggggctccctttagggttccgatttagtgctttacggcacctcgaccccaaaaaacttgattagggtgatggttcacgtagtgggccatcgccctgatagacggtttttcgccctttgacgttggagtccacgttctttaatagtggactcttgttccaaactggaacaacactcaaccctatctcggtctattcttttgatttataagggattttgccgatttcggcctattggttaaaaaatgagctgatttaacaaaaatttaacgcgaattaattctgtggaatgtgtgtcagttagtcgcgatgtgtgactagttagttattaatagtaatcaattacggggtcattagttcatagcccatatatggagttccgcgttacataacttacggtaaatggcccgcctggctgaccgcccaacgacccccgcccattgacgtcaataatgacgtatgttcccatagtaacgccaatagggactttccattgacgtcaatgggtggagtatttacggtaaactgcccacttggcagtacatcaagtgtatcatatgccaagtacgccccctattgacgtcaatgacggtaaatggcccgcctggcattatgcccagtacatgaccttatgggactttcctacttggcagtacatctacgtattagtcatcgctattaccatggtgatgcggttttggcagtacatcaatgggcgtggatagcggtttgactcacggggatttccaagtctccaccccattgacgtcaatgggagtttgttttggcaccaaaatcaacgggactttccaaaatgtcgtaacaactccgccccattgacgcaaatgggcggtaggcgtgtacggtgggaggtctatataagcagagctcatgatagaagcactctactattcgtcgaccgatcctgagaacttcagggtgagtttggggacccttgattgttctttctttttcgctattgtaaaattcatgttatatggagggggcaaagttttcagggtgttgtttagaatgggaagatgtcccttgtatcaccatggaccctcatgataattttgtttctttcactttctactctgttgacaaccattgtctcctcttattttcttttcattttctgtaactttttcgttaaactttagcttgcatttgtaacgaatttttaaattcacttttgtttatttgtcagattgtaagtactttctctaatcacttttttttcaaggcaatcagggtatattatattgtacttcagcacagttttagagaacaattgttataattaaatgataaggtagaatatttctgcatataaattctggctggcgtggaaatattcttattggtagaaacaactacaccctggtcatcatcctgcctttctctttatggttacaatgatatacactgtttgagatgaggataaaatactctgagtccaaaccgggcccctctgctaaccatgttcatgccttcttctctttcctacagctcctgggcaacgtgctggttgttgtgctgtctcatcattttggcaaagaattaagcttatac

SEQ ID NO: 43 - protein, 115 aa, Artificial
  consensus sequence
  MISC_FEATURE (1)..(1): Xaa can be any naturally occurring amino acid
  MISC_FEATURE (11)..(11): Xaa can be any naturally occurring amino acid
  MISC_FEATURE (28)..(28): Xaa can be any naturally occurring amino acid
  MISC_FEATURE (30)..(30): Xaa can be any naturally occurring amino acid
  MISC_FEATURE (34)..(35): Xaa can be any naturally occurring amino acid
  MISC_FEATURE (93)..(93): Xaa can be any naturally occurring amino acid
  MISC_FEATURE (93)..(93): Xaa can be any naturally occurring amino acid
  MISC_FEATURE (96)..(96): Xaa can be any naturally occurring amino acid
  MISC_FEATURE (100)..(100): Xaa can be any naturally occurring amino acid
  misc_feature (111)..(111): Xaa can be any naturally occurring amino acid
  MISC_FEATURE (114)..(114): Xaa can be any naturally occurring amino acid
XDVWGQGTTVXVSSASTKGPSVFPLAPXSXSTSXXTAALGCLVKDYFPEPVTVSWNSGALTSGVHTFPAVLQSSGLYSLSSVVTVPSSSLGTXTYXCNVXHKPSNTKVDKXVEXK

SEQ ID NO: 44 - protein, 225 aa, Artificial
  consensus sequence
  MISC_FEATURE (13)..(13): Xaa can be any naturally occurring amino acid
  MISC_FEATURE (47)..(47): Xaa can be any naturally occurring amino acid
  MISC_FEATURE (53)..(53): Xaa can be any naturally occurring amino acid
  MISC_FEATURE (75)..(75): Xaa can be any naturally occurring amino acid
  MISC_FEATURE (106)..(106): Xaa can be any naturally occurring amino acid
  MISC_FEATURE (109)..(110): Xaa can be any naturally occurring amino acid
  MISC_FEATURE (134)..(135): Xaa can be any naturally occurring amino acid
  misc_feature (137)..(137): Xaa can be any naturally occurring amino acid
  MISC_FEATURE (188)..(188): Xaa can be any naturally occurring amino acid
  MISC_FEATURE (198)..(198): Xaa can be any naturally occurring amino acid
  MISC_FEATURE (224)..(224): Xaa can be any naturally occurring amino acid
YGPPCPPCPAPEXLGGPSVFLFPPKPKDTLMISRTPEVTCVVVDVSXEDPEVXFNWYVDGVEVHNAKTKPREEQXNSTYRVVSVLTVLHQDWLNGKEYKCKVSNKXLPXXIEKTISKAKGQPREPQVYTLPPSXXEXTKNQVSLTCLVKGFYPSDIAVEWESNGQPENNYKTTPPVLDSDGSFFLYSXLTVDKSRWQXGNVFSCSVMHEALHNHYTQKSLSLSXG

SEQ ID NO: 45 - protein, 60 aa, Artificial
  consensus sequence
  MISC_FEATURE (13)..(14): Xaa can be any naturally occurring amino acid
  MISC_FEATURE (16)..(16): Xaa can be any naturally occurring amino acid
  MISC_FEATURE (21)..(22): Xaa can be any naturally occurring amino acid
  MISC_FEATURE (24)..(27): Xaa can be any naturally occurring amino acid
  MISC_FEATURE (31)..(31): Xaa can be any naturally occurring amino acid
  MISC_FEATURE (34)..(34): Xaa can be any naturally occurring amino acid
  MISC_FEATURE (48)..(48): Xaa can be any naturally occurring amino acid
  misc_feature (50)..(50): Xaa can be any naturally occurring amino acid
  MISC_FEATURE (54)..(54): Xaa can be any naturally occurring amino acid
  MISC_FEATURE (56)..(56): Xaa can be any naturally occurring amino acid
SDYLAWYQQKPGXXPXLLIYXXSXXXXGVPXRFXGSGSGTDFTLTISXLXPEDXAXYYCQ

SEQ ID NO: 46 - protein, 118 aa, Artificial
  consensus sequence
  MISC_FEATURE (4)..(4): Xaa can be any naturally occurring amino acid
TFGXGTKVEIKRTVAAPSVFIFPPSDEQLKSGTASVVCLLNNFYPREAKVQWKVDNALQSGNSQESVTEQDSKDSTYSLSSTLTLSKADYEKHKVYACEVTHQGLSSPVTKSFNRGEC